European Patent Specification EP 3 341 395 B1, published November 29, 2023. Title: Improved Cell-Permeable (iCP)-SOCS3 Recombinant Protein and Uses Thereof. Applicant: Daewoong Jo Cellivery Therapeutics, Inc. The sequence listing filed with the application follows.

SEQUENCE LISTING (831 sequences)

SEQ ID NO: 1 - protein, 12 aa, Artificial Sequence
  Amino acid Sequence of aMTD1
AAALAPVVLALP

SEQ ID NO: 2 - protein, 12 aa, Artificial Sequence
  Amino acid Sequence of aMTD2
AAAVPLLAVVVP

SEQ ID NO: 3 - protein, 12 aa, Artificial Sequence
  Amino acid Sequence of aMTD3
AALLVPAAVLAP

SEQ ID NO: 4 - protein, 12 aa, Artificial Sequence
  Amino acid Sequence of aMTD4
ALALLPVAALAP

SEQ ID NO: 5 - protein, 12 aa, Artificial Sequence
  Amino acid Sequence of aMTD5
AAALLPVALVAP

SEQ ID NO: 6 - protein, 12 aa, Artificial Sequence
  Amino acid Sequence of aMTD11
VVALAPALAALP

SEQ ID NO: 7 - protein, 12 aa, Artificial Sequence
  Amino acid Sequence of aMTD12
LLAAVPAVLLAP

SEQ ID NO: 8 - protein, 12 aa, Artificial Sequence
  Amino acid Sequence of aMTD13
AAALVPVVALLP

SEQ ID NO: 9 - protein, 12 aa, Artificial Sequence
  Amino acid Sequence of aMTD21
AVALLPALLAVP

SEQ ID NO: 10 - protein, 12 aa, Artificial Sequence
  Amino acid Sequence of aMTD22
AVVLVPVLAAAP

SEQ ID NO: 11 - protein, 12 aa, Artificial Sequence
  Amino acid Sequence of aMTD23
VVLVLPAAAAVP

SEQ ID NO: 12 - protein, 12 aa, Artificial Sequence
  Amino acid Sequence of aMTD24
IALAAPALIVAP

SEQ ID NO: 13 - protein, 12 aa, Artificial Sequence
  Amino acid Sequence of aMTD25
IVAVAPALVALP

SEQ ID NO: 14 - protein, 12 aa, Artificial Sequence
  Amino acid Sequence of aMTD42
VAALPVVAVVAP

SEQ ID NO: 15 - protein, 12 aa, Artificial Sequence
  Amino acid Sequence of aMTD43
LLAAPLVVAAVP

SEQ ID NO: 16 - protein, 12 aa, Artificial Sequence
  Amino acid Sequence of aMTD44
ALAVPVALLVAP

SEQ ID NO: 17 - protein, 12 aa, Artificial Sequence
  Amino acid Sequence of aMTD61
VAALPVLLAALP

SEQ ID NO: 18 - protein, 12 aa, Artificial Sequence
  Amino acid Sequence of aMTD62
VALLAPVALAVP

SEQ ID NO: 19 - protein, 12 aa, Artificial Sequence
  Amino acid Sequence of aMTD63
AALLVPALVAVP

SEQ ID NO: 20 - protein, 12 aa, Artificial Sequence
  Amino acid Sequence of aMTD64
AIVALPVAVLAP

SEQ ID NO: 21 - protein, 12 aa, Artificial Sequence
  Amino acid Sequence of aMTD65
IAIVAPVVALAP

SEQ ID NO: 22 - protein, 12 aa, Artificial Sequence
  Amino acid Sequence of aMTD81
AALLPALAALLP

SEQ ID NO: 23 - protein, 12 aa, Artificial Sequence
  Amino acid Sequence of aMTD82
AVVLAPVAAVLP

SEQ ID NO: 24 - protein, 12 aa, Artificial Sequence
  Amino acid Sequence of aMTD83
LAVAAPLALALP

SEQ ID NO: 25 - protein, 12 aa, Artificial Sequence
  Amino acid Sequence of aMTD84
AAVAAPLLLALP

SEQ ID NO: 26 - protein, 12 aa, Artificial Sequence
  Amino acid Sequence of aMTD85
LLVLPAAALAAP

SEQ ID NO: 27 - protein, 12 aa, Artificial Sequence
  Amino acid Sequence of aMTD101
LVALAPVAAVLP

SEQ ID NO: 28 - protein, 12 aa, Artificial Sequence
  Amino acid Sequence of aMTD102
LALAPAALALLP

SEQ ID NO: 29 - protein, 12 aa, Artificial Sequence
  Amino acid Sequence of aMTD103
ALIAAPILALAP

SEQ ID NO: 30 - protein, 12 aa, Artificial Sequence
  Amino acid Sequence of aMTD104
AVVAAPLVLALP

SEQ ID NO: 31 - protein, 12 aa, Artificial Sequence
  Amino acid Sequence of aMTD105
LLALAPAALLAP

SEQ ID NO: 32 - protein, 12 aa, Artificial Sequence
  Amino acid Sequence of aMTD121
AIVALPALALAP

SEQ ID NO: 33 - protein, 12 aa, Artificial Sequence
  Amino acid Sequence of aMTD123
AAIIVPAALLAP

SEQ ID NO: 34 - protein, 12 aa, Artificial Sequence
  Amino acid Sequence of aMTD124
IAVALPALIAAP

SEQ ID NO: 35 - protein, 12 aa, Artificial Sequence
  Amino acid Sequence of aMTD141
AVIVLPALAVAP

SEQ ID NO: 36 - protein, 12 aa, Artificial Sequence
  Amino acid Sequence of aMTD143
AVLAVPAVLVAP

SEQ ID NO: 37 - protein, 12 aa, Artificial Sequence
  Amino acid Sequence of aMTD144
VLAIVPAVALAP

SEQ ID NO: 38 - protein, 12 aa, Artificial Sequence
  Amino acid Sequence of aMTD145
LLAVVPAVALAP

SEQ ID NO: 39 - protein, 12 aa, Artificial Sequence
  Amino acid Sequence of aMTD161
AVIALPALIAAP

SEQ ID NO: 40 - protein, 12 aa, Artificial Sequence
  Amino acid Sequence of aMTD162
AVVALPAALIVP

SEQ ID NO: 41 - protein, 12 aa, Artificial Sequence
  Amino acid Sequence of aMTD163
LALVLPAALAAP

SEQ ID NO: 42 - protein, 12 aa, Artificial Sequence
  Amino acid Sequence of aMTD164
LAAVLPALLAAP

SEQ ID NO: 43 - protein, 12 aa, Artificial Sequence
  Amino acid Sequence of aMTD165
ALAVPVALAIVP

SEQ ID NO: 44 - protein, 12 aa, Artificial Sequence
  Amino acid Sequence of aMTD182
ALIAPVVALVAP

SEQ ID NO: 45 - protein, 12 aa, Artificial Sequence
  Amino acid Sequence of aMTD183
LLAAPVVIALAP

SEQ ID NO: 46 - protein, 12 aa, Artificial Sequence
  Amino acid Sequence of aMTD184
LAAIVPAIIAVP

SEQ ID NO: 47 - protein, 12 aa, Artificial Sequence
  Amino acid Sequence of aMTD185
AALVLPLIIAAP

SEQ ID NO: 48 - protein, 12 aa, Artificial Sequence
  Amino acid Sequence of aMTD201
LALAVPALAALP

SEQ ID NO: 49 - protein, 12 aa, Artificial Sequence
  Amino acid Sequence of aMTD204
LIAALPAVAALP

SEQ ID NO: 50 - protein, 12 aa, Artificial Sequence
  Amino acid Sequence of aMTD205
ALALVPAIAALP

SEQ ID NO: 51 - protein, 12 aa, Artificial Sequence
  Amino acid Sequence of aMTD221
AAILAPIVALAP

SEQ ID NO: 52 - protein, 12 aa, Artificial Sequence
  Amino acid Sequence of aMTD222
ALLIAPAAVIAP

SEQ ID NO: 53 - protein, 12 aa, Artificial Sequence
  Amino acid Sequence of aMTD223
AILAVPIAVVAP

SEQ ID NO: 54 - protein, 12 aa, Artificial Sequence
  Amino acid Sequence of aMTD224
ILAAVPIALAAP

SEQ ID NO: 55 - protein, 12 aa, Artificial Sequence
  Amino acid Sequence of aMTD225
VAALLPAAAVLP

SEQ ID NO: 56 - protein, 12 aa, Artificial Sequence
  Amino acid Sequence of aMTD241
AAAVVPVLLVAP

SEQ ID NO: 57 - protein, 12 aa, Artificial Sequence
  Amino acid Sequence of aMTD242
AALLVPALVAAP

SEQ ID NO: 58 - protein, 12 aa, Artificial Sequence
  Amino acid Sequence of aMTD243
AAVLLPVALAAP

SEQ ID NO: 59 - protein, 12 aa, Artificial Sequence
  Amino acid Sequence of aMTD245
AAALAPVLALVP

SEQ ID NO: 60 - protein, 12 aa, Artificial Sequence
  Amino acid Sequence of aMTD261
LVLVPLLAAAAP

SEQ ID NO: 61 - protein, 12 aa, Artificial Sequence
  Amino acid Sequence of aMTD262
ALIAVPAIIVAP

SEQ ID NO: 62 - protein, 12 aa, Artificial Sequence
  Amino acid Sequence of aMTD263
ALAVIPAAAILP

SEQ ID NO: 63 - protein, 12 aa, Artificial Sequence
  Amino acid Sequence of aMTD264
LAAAPVVIVIAP

SEQ ID NO: 64 - protein, 12 aa, Artificial Sequence
  Amino acid Sequence of aMTD265
VLAIAPLLAAVP

SEQ ID NO: 65 - protein, 12 aa, Artificial Sequence
  Amino acid Sequence of aMTD281
ALIVLPAAVAVP

SEQ ID NO: 66 - protein, 12 aa, Artificial Sequence
  Amino acid Sequence of aMTD282
VLAVAPALIVAP

SEQ ID NO: 67 - protein, 12 aa, Artificial Sequence
  Amino acid Sequence of aMTD283
AALLAPALIVAP

SEQ ID NO: 68 - protein, 12 aa, Artificial Sequence
  Amino acid Sequence of aMTD284
ALIAPAVALIVP

SEQ ID NO: 69 - protein, 12 aa, Artificial Sequence
  Amino acid Sequence of aMTD285
AIVLLPAAVVAP

SEQ ID NO: 70 - protein, 12 aa, Artificial Sequence
  Amino acid Sequence of aMTD301
VIAAPVLAVLAP

SEQ ID NO: 71 - protein, 12 aa, Artificial Sequence
  Amino acid Sequence of aMTD302
LALAPALALLAP

SEQ ID NO: 72 - protein, 12 aa, Artificial Sequence
  Amino acid Sequence of aMTD304
AIILAPIAAIAP

SEQ ID NO: 73 - protein, 12 aa, Artificial Sequence
  Amino acid Sequence of aMTD305
IALAAPILLAAP

SEQ ID NO: 74 - protein, 12 aa, Artificial Sequence
  Amino acid Sequence of aMTD321
IVAVALPALAVP

SEQ ID NO: 75 - protein, 12 aa, Artificial Sequence
  Amino acid Sequence of aMTD322
VVAIVLPALAAP

SEQ ID NO: 76 - protein, 12 aa, Artificial Sequence
  Amino acid Sequence of aMTD323
IVAVALPVALAP

SEQ ID NO: 77 - protein, 12 aa, Artificial Sequence
  Amino acid Sequence of aMTD324
IVAVALPAALVP

SEQ ID NO: 78 - protein, 12 aa, Artificial Sequence
  Amino acid Sequence of aMTD325
IVAVALPAVALP

SEQ ID NO: 79 - protein, 12 aa, Artificial Sequence
  Amino acid Sequence of aMTD341
IVAVALPAVLAP

SEQ ID NO: 80 - protein, 12 aa, Artificial Sequence
  Amino acid Sequence of aMTD342
VIVALAPAVLAP

SEQ ID NO: 81 - protein, 12 aa, Artificial Sequence
  Amino acid Sequence of aMTD343
IVAVALPALVAP

SEQ ID NO: 82 - protein, 12 aa, Artificial Sequence
  Amino acid Sequence of aMTD345
ALLIVAPVAVAP

SEQ ID NO: 83 - protein, 12 aa, Artificial Sequence
  Amino acid Sequence of aMTD361
AVVIVAPAVIAP

SEQ ID NO: 84 - protein, 12 aa, Artificial Sequence
  Amino acid Sequence of aMTD363
AVLAVAPALIVP

SEQ ID NO: 85 - protein, 12 aa, Artificial Sequence
  Amino acid Sequence of aMTD364
LVAAVAPALIVP

SEQ ID NO: 86 - protein, 12 aa, Artificial Sequence
  Amino acid Sequence of aMTD365
AVIVVAPALLAP

SEQ ID NO: 87 - protein, 12 aa, Artificial Sequence
  Amino acid Sequence of aMTD381
VVAIVLPAVAAP

SEQ ID NO: 88 - protein, 12 aa, Artificial Sequence
  Amino acid Sequence of aMTD382
AAALVIPAILAP

SEQ ID NO: 89 - protein, 12 aa, Artificial Sequence
  Amino acid Sequence of aMTD383
VIVALAPALLAP

SEQ ID NO: 90 - protein, 12 aa, Artificial Sequence
  Amino acid Sequence of aMTD384
VIVAIAPALLAP

SEQ ID NO: 91 - protein, 12 aa, Artificial Sequence
  Amino acid Sequence of aMTD385
IVAIAVPALVAP

SEQ ID NO: 92 - protein, 12 aa, Artificial Sequence
  Amino acid Sequence of aMTD401
AALAVIPAAILP

SEQ ID NO: 93 - protein, 12 aa, Artificial Sequence
  Amino acid Sequence of aMTD402
ALAAVIPAAILP

SEQ ID NO: 94 - protein, 12 aa, Artificial Sequence
  Amino acid Sequence of aMTD403
AAALVIPAAILP

SEQ ID NO: 95 - protein, 12 aa, Artificial Sequence
  Amino acid Sequence of aMTD404
LAAAVIPAAILP

SEQ ID NO: 96 - protein, 12 aa, Artificial Sequence
  Amino acid Sequence of aMTD405
LAAAVIPVAILP

SEQ ID NO: 97 - protein, 12 aa, Artificial Sequence
  Amino acid Sequence of aMTD421
AAILAAPLIAVP

SEQ ID NO: 98 - protein, 12 aa, Artificial Sequence
  Amino acid Sequence of aMTD422
VVAILAPLLAAP

SEQ ID NO: 99 - protein, 12 aa, Artificial Sequence
  Amino acid Sequence of aMTD424
AVVVAAPVLALP

SEQ ID NO: 100 - protein, 12 aa, Artificial Sequence
  Amino acid Sequence of aMTD425
AVVAIAPVLALP

SEQ ID NO: 101 - protein, 12 aa, Artificial Sequence
  Amino acid Sequence of aMTD442
ALAALVPAVLVP

SEQ ID NO: 102 - protein, 12 aa, Artificial Sequence
  Amino acid Sequence of aMTD443
ALAALVPVALVP

SEQ ID NO: 103 - protein, 12 aa, Artificial Sequence
  Amino acid Sequence of aMTD444
LAAALVPVALVP

SEQ ID NO: 104 - protein, 12 aa, Artificial Sequence
  Amino acid Sequence of aMTD445
ALAALVPALVVP

SEQ ID NO: 105 - protein, 12 aa, Artificial Sequence
  Amino acid Sequence of aMTD461
IAAVIVPAVALP

SEQ ID NO: 106 - protein, 12 aa, Artificial Sequence
  Amino acid Sequence of aMTD462
IAAVLVPAVALP

SEQ ID NO: 107 - protein, 12 aa, Artificial Sequence
  Amino acid Sequence of aMTD463
AVAILVPLLAAP

SEQ ID NO: 108 - protein, 12 aa, Artificial Sequence
  Amino acid Sequence of aMTD464
AVVILVPLAAAP

SEQ ID NO: 109 - protein, 12 aa, Artificial Sequence
  Amino acid Sequence of aMTD465
IAAVIVPVAALP

SEQ ID NO: 110 - protein, 12 aa, Artificial Sequence
  Amino acid Sequence of aMTD481
AIAIAIVPVALP

SEQ ID NO: 111 - protein, 12 aa, Artificial Sequence
  Amino acid Sequence of aMTD482
ILAVAAIPVAVP

SEQ ID NO: 112 - protein, 12 aa, Artificial Sequence
  Amino acid Sequence of aMTD483
ILAAAIIPAALP

SEQ ID NO: 113 - protein, 12 aa, Artificial Sequence
  Amino acid Sequence of aMTD484
LAVVLAAPAIVP

SEQ ID NO: 114 - protein, 12 aa, Artificial Sequence
  Amino acid Sequence of aMTD485
AILAAIVPLAVP

SEQ ID NO: 115 - protein, 12 aa, Artificial Sequence
  Amino acid Sequence of aMTD501
VIVALAVPALAP

SEQ ID NO: 116 - protein, 12 aa, Artificial Sequence
  Amino acid Sequence of aMTD502
AIVALAVPVLAP

SEQ ID NO: 117 - protein, 12 aa, Artificial Sequence
  Amino acid Sequence of aMTD503
AAIIIVLPAALP

SEQ ID NO: 118 - protein, 12 aa, Artificial Sequence
  Amino acid Sequence of aMTD504
LIVALAVPALAP

SEQ ID NO: 119 - protein, 12 aa, Artificial Sequence
  Amino acid Sequence of aMTD505
AIIIVIAPAAAP

SEQ ID NO: 120 - protein, 12 aa, Artificial Sequence
  Amino acid Sequence of aMTD521
LAALIVVPAVAP

SEQ ID NO: 121 - protein, 12 aa, Artificial Sequence
  Amino acid Sequence of aMTD522
ALLVIAVPAVAP

SEQ ID NO: 122 - protein, 12 aa, Artificial Sequence
  Amino acid Sequence of aMTD524
AVALIVVPALAP

SEQ ID NO: 123 - protein, 12 aa, Artificial Sequence
  Amino acid Sequence of aMTD525
ALAIVVAPVAVP

SEQ ID NO: 124 - protein, 12 aa, Artificial Sequence
  Amino acid Sequence of aMTD541
LLALIIAPAAAP

SEQ ID NO: 125 - protein, 12 aa, Artificial Sequence
  Amino acid Sequence of aMTD542
ALALIIVPAVAP

SEQ ID NO: 126 - protein, 12 aa, Artificial Sequence
  Amino acid Sequence of aMTD543
LLAALIAPAALP

SEQ ID NO: 127 - protein, 12 aa, Artificial Sequence
  Amino acid Sequence of aMTD544
IVALIVAPAAVP

SEQ ID NO: 128 - protein, 12 aa, Artificial Sequence
  Amino acid Sequence of aMTD545
VVLVLAAPAAVP

SEQ ID NO: 129 - protein, 12 aa, Artificial Sequence
  Amino acid Sequence of aMTD561
AAVAIVLPAVVP

SEQ ID NO: 130 - protein, 12 aa, Artificial Sequence
  Amino acid Sequence of aMTD562
ALIAAIVPALVP

SEQ ID NO: 131 - protein, 12 aa, Artificial Sequence
  Amino acid Sequence of aMTD563
ALAVIVVPALAP

SEQ ID NO: 132 - protein, 12 aa, Artificial Sequence
  Amino acid Sequence of aMTD564
VAIALIVPALAP

SEQ ID NO: 133 - protein, 12 aa, Artificial Sequence
  Amino acid Sequence of aMTD565
VAIVLVAPAVAP

SEQ ID NO: 134 - protein, 12 aa, Artificial Sequence
  Amino acid Sequence of aMTD582
VAVALIVPALAP

SEQ ID NO: 135 - protein, 12 aa, Artificial Sequence
  Amino acid Sequence of aMTD583
AVILALAPIVAP

SEQ ID NO: 136 - protein, 12 aa, Artificial Sequence
  Amino acid Sequence of aMTD585
ALIVAIAPALVP

SEQ ID NO: 137 - protein, 12 aa, Artificial Sequence
  Amino acid Sequence of aMTD601
AAILIAVPIAAP

SEQ ID NO: 138 - protein, 12 aa, Artificial Sequence
  Amino acid Sequence of aMTD602
VIVALAAPVLAP

SEQ ID NO: 139 - protein, 12 aa, Artificial Sequence
  Amino acid Sequence of aMTD603
VLVALAAPVIAP

SEQ ID NO: 140 - protein, 12 aa, Artificial Sequence
  Amino acid Sequence of aMTD604
VALIAVAPAVVP

SEQ ID NO: 141 - protein, 12 aa, Artificial Sequence
  Amino acid Sequence of aMTD605
VIAAVLAPVAVP

SEQ ID NO: 142 - protein, 12 aa, Artificial Sequence
  Amino acid Sequence of aMTD622
ALIVLAAPVAVP

SEQ ID NO: 143 - protein, 12 aa, Artificial Sequence
  Amino acid Sequence of aMTD623
VAAAIALPAIVP

SEQ ID NO: 144 - protein, 12 aa, Artificial Sequence
  Amino acid Sequence of aMTD625
ILAAAAAPLIVP

SEQ ID NO: 145 - protein, 12 aa, Artificial Sequence
  Amino acid Sequence of aMTD643
LALVLAAPAIVP

SEQ ID NO: 146 - protein, 12 aa, Artificial Sequence
  Amino acid Sequence of aMTD645
ALAVVALPAIVP

SEQ ID NO: 147 - protein, 12 aa, Artificial Sequence
  Amino acid Sequence of aMTD661
AAILAPIVAALP

SEQ ID NO: 148 - protein, 12 aa, Artificial Sequence
  Amino acid Sequence of aMTD664
ILIAIAIPAAAP

SEQ ID NO: 149 - protein, 12 aa, Artificial Sequence
  Amino acid Sequence of aMTD665
LAIVLAAPVAVP

SEQ ID NO: 150 - protein, 12 aa, Artificial Sequence
  Amino acid Sequence of aMTD666
AAIAIIAPAIVP

SEQ ID NO: 151 - protein, 12 aa, Artificial Sequence
  Amino acid Sequence of aMTD667
LAVAIVAPALVP

SEQ ID NO: 152 - protein, 12 aa, Artificial Sequence
  Amino acid Sequence of aMTD683
LAIVLAAPAVLP

SEQ ID NO: 153 - protein, 12 aa, Artificial Sequence
  Amino acid Sequence of aMTD684
AAIVLALPAVLP

SEQ ID NO: 154 - protein, 12 aa, Artificial Sequence
  Amino acid Sequence of aMTD685
ALLVAVLPAALP

SEQ ID NO: 155 - protein, 12 aa, Artificial Sequence
  Amino acid Sequence of aMTD686
AALVAVLPVALP

SEQ ID NO: 156 - protein, 12 aa, Artificial Sequence
  Amino acid Sequence of aMTD687
AILAVALPLLAP

SEQ ID NO: 157 - protein, 12 aa, Artificial Sequence
  Amino acid Sequence of aMTD703
IVAVALVPALAP

SEQ ID NO: 158 - protein, 12 aa, Artificial Sequence
  Amino acid Sequence of aMTD705
IVAVALLPALAP

SEQ ID NO: 159 - protein, 12 aa, Artificial Sequence
  Amino acid Sequence of aMTD706
IVAVALLPAVAP

SEQ ID NO: 160 - protein, 12 aa, Artificial Sequence
  Amino acid Sequence of aMTD707
IVALAVLPAVAP

SEQ ID NO: 161 - protein, 12 aa, Artificial Sequence
  Amino acid Sequence of aMTD724
VAVLAVLPALAP

SEQ ID NO: 162 - protein, 12 aa, Artificial Sequence
  Amino acid Sequence of aMTD725
IAVLAVAPAVLP

SEQ ID NO: 163 - protein, 12 aa, Artificial Sequence
  Amino acid Sequence of aMTD726
LAVAIIAPAVAP

SEQ ID NO: 164 - protein, 12 aa, Artificial Sequence
  Amino acid Sequence of aMTD727
VALAIALPAVLP

SEQ ID NO: 165 - protein, 12 aa, Artificial Sequence
  Amino acid Sequence of aMTD743
AIAIALVPVALP

SEQ ID NO: 166 - protein, 12 aa, Artificial Sequence
  Amino acid Sequence of aMTD744
AAVVIVAPVALP

SEQ ID NO: 167 - protein, 12 aa, Artificial Sequence
  Amino acid Sequence of aMTD746
VAIIVVAPALAP

SEQ ID NO: 168 - protein, 12 aa, Artificial Sequence
  Amino acid Sequence of aMTD747
VALLAIAPALAP

SEQ ID NO: 169 - protein, 12 aa, Artificial Sequence
  Amino acid Sequence of aMTD763
VAVLIAVPALAP

SEQ ID NO: 170 - protein, 12 aa, Artificial Sequence
  Amino acid Sequence of aMTD764
AVALAVLPAVVP

SEQ ID NO: 171 - protein, 12 aa, Artificial Sequence
  Amino acid Sequence of aMTD765
AVALAVVPAVLP

SEQ ID NO: 172 - protein, 12 aa, Artificial Sequence
  Amino acid Sequence of aMTD766
IVVIAVAPAVAP

SEQ ID NO: 173 - protein, 12 aa, Artificial Sequence
  Amino acid Sequence of aMTD767
IVVAAVVPALAP

SEQ ID NO: 174 - protein, 12 aa, Artificial Sequence
  Amino acid Sequence of aMTD783
IVALVPAVAIAP

SEQ ID NO: 175 - protein, 12 aa, Artificial Sequence
  Amino acid Sequence of aMTD784
VAALPAVALVVP

SEQ ID NO: 176 - protein, 12 aa, Artificial Sequence
  Amino acid Sequence of aMTD786
LVAIAPLAVLAP

SEQ ID NO: 177 - protein, 12 aa, Artificial Sequence
  Amino acid Sequence of aMTD787
AVALVPVIVAAP

SEQ ID NO: 178 - protein, 12 aa, Artificial Sequence
  Amino acid Sequence of aMTD788
AIAVAIAPVALP

SEQ ID NO: 179 - protein, 12 aa, Artificial Sequence
  Amino acid Sequence of aMTD803
AIALAVPVLALP

SEQ ID NO: 180 - protein, 12 aa, Artificial Sequence
  Amino acid Sequence of aMTD805
LVLIAAAPIALP

SEQ ID NO: 181 - protein, 12 aa, Artificial Sequence
  Amino acid Sequence of aMTD806
LVALAVPAAVLP

SEQ ID NO: 182 - protein, 12 aa, Artificial Sequence
  Amino acid Sequence of aMTD807
AVALAVPALVLP

SEQ ID NO: 183 - protein, 12 aa, Artificial Sequence
  Amino acid Sequence of aMTD808
LVVLAAAPLAVP

SEQ ID NO: 184 - protein, 12 aa, Artificial Sequence
  Amino acid Sequence of aMTD809
LIVLAAPALAAP

SEQ ID NO: 185 - protein, 12 aa, Artificial Sequence
  Amino acid Sequence of aMTD810
VIVLAAPALAAP

SEQ ID NO: 186 - protein, 12 aa, Artificial Sequence
  Amino acid Sequence of aMTD811
AVVLAVPALAVP

SEQ ID NO: 187 - protein, 12 aa, Artificial Sequence
  Amino acid Sequence of aMTD824
LIIVAAAPAVAP

SEQ ID NO: 188 - protein, 12 aa, Artificial Sequence
  Amino acid Sequence of aMTD825
IVAVIVAPAVAP

SEQ ID NO: 189 - protein, 12 aa, Artificial Sequence
  Amino acid Sequence of aMTD826
LVALAAPIIAVP

SEQ ID NO: 190 - protein, 12 aa, Artificial Sequence
  Amino acid Sequence of aMTD827
IAAVLAAPALVP

SEQ ID NO: 191 - protein, 12 aa, Artificial Sequence
  Amino acid Sequence of aMTD828
IALLAAPIIAVP

SEQ ID NO: 192 - protein, 12 aa, Artificial Sequence
  Amino acid Sequence of aMTD829
AALALVAPVIVP

SEQ ID NO: 193 - protein, 12 aa, Artificial Sequence
  Amino acid Sequence of aMTD830
IALVAAPVALVP

SEQ ID NO: 194 - protein, 12 aa, Artificial Sequence
  Amino acid Sequence of aMTD831
IIVAVAPAAIVP

SEQ ID NO: 195 - protein, 12 aa, Artificial Sequence
  Amino acid Sequence of aMTD832
AVAAIVPVIVAP

SEQ ID NO: 196 - protein, 12 aa, Artificial Sequence
  Amino acid Sequence of aMTD843
AVLVLVAPAAAP

SEQ ID NO: 197 - protein, 12 aa, Artificial Sequence
  Amino acid Sequence of aMTD844
VVALLAPLIAAP

SEQ ID NO: 198 - protein, 12 aa, Artificial Sequence
  Amino acid Sequence of aMTD845
AAVVIAPLLAVP

SEQ ID NO: 199 - protein, 12 aa, Artificial Sequence
  Amino acid Sequence of aMTD846
IAVAVAAPLLVP

SEQ ID NO: 200 - protein, 12 aa, Artificial Sequence
  Amino acid Sequence of aMTD847
LVAIVVLPAVAP

SEQ ID NO: 201 - protein, 12 aa, Artificial Sequence
  Amino acid Sequence of aMTD848
AVAIVVLPAVAP

SEQ ID NO: 202 - protein, 12 aa, Artificial Sequence
  Amino acid Sequence of aMTD849
AVILLAPLIAAP

SEQ ID NO: 203 - protein, 12 aa, Artificial Sequence
  Amino acid Sequence of aMTD850
LVIALAAPVALP

SEQ ID NO: 204 - protein, 12 aa, Artificial Sequence
  Amino acid Sequence of aMTD851
VLAVVLPAVALP

SEQ ID NO: 205 - protein, 12 aa, Artificial Sequence
  Amino acid Sequence of aMTD852
VLAVAAPAVLLP

SEQ ID NO: 206 - protein, 12 aa, Artificial Sequence
  Amino acid Sequence of aMTD863
AAVVLLPIIAAP

SEQ ID NO: 207 - protein, 12 aa, Artificial Sequence
  Amino acid Sequence of aMTD864
ALLVIAPAIAVP

SEQ ID NO: 208 - protein, 12 aa, Artificial Sequence
  Amino acid Sequence of aMTD865
AVLVIAVPAIAP

SEQ ID NO: 209 - protein, 12 aa, Artificial Sequence
  Amino acid Sequence of aMTD867
ALLVVIAPLAAP

SEQ ID NO: 210 - protein, 12 aa, Artificial Sequence
  Amino acid Sequence of aMTD868
VLVAAILPAAIP

SEQ ID NO: 211 - protein, 12 aa, Artificial Sequence
  Amino acid Sequence of aMTD870
VLVAAVLPIAAP

SEQ ID NO: 212 - protein, 12 aa, Artificial Sequence
  Amino acid Sequence of aMTD872
VLAAAVLPLVVP

SEQ ID NO: 213 - protein, 12 aa, Artificial Sequence
  Amino acid Sequence of aMTD875
AIAIVVPAVAVP

SEQ ID NO: 214 - protein, 12 aa, Artificial Sequence
  Amino acid Sequence of aMTD877
VAIIAVPAVVAP

SEQ ID NO: 215 - protein, 12 aa, Artificial Sequence
  Amino acid Sequence of aMTD878
IVALVAPAAVVP

SEQ ID NO: 216 - protein, 12 aa, Artificial Sequence
  Amino acid Sequence of aMTD879
AAIVLLPAVVVP

SEQ ID NO: 217 - protein, 12 aa, Artificial Sequence
  Amino acid Sequence of aMTD881
AALIVVPAVAVP

SEQ ID NO: 218 - protein, 12 aa, Artificial Sequence
  Amino acid Sequence of aMTD882
AIALVVPAVAVP

SEQ ID NO: 219 - protein, 12 aa, Artificial Sequence
  Amino acid Sequence of aMTD883
LAIVPAAIAALP

SEQ ID NO: 220 - protein, 12 aa, Artificial Sequence
  Amino acid Sequence of aMTD885
LVAIAPAVAVLP

SEQ ID NO: 221 - protein, 12 aa, Artificial Sequence
  Amino acid Sequence of aMTD887
VLAVAPAVAVLP

SEQ ID NO: 222 - protein, 12 aa, Artificial Sequence
  Amino acid Sequence of aMTD888
ILAVVAIPAAAP

SEQ ID NO: 223 - protein, 12 aa, Artificial Sequence
  Amino acid Sequence of aMTD889
ILVAAAPIAALP

SEQ ID NO: 224 - protein, 12 aa, Artificial Sequence
  Amino acid Sequence of aMTD891
ILAVAAIPAALP

SEQ ID NO: 225 - protein, 12 aa, Artificial Sequence
  Amino acid Sequence of aMTD893
VIAIPAILAAAP

SEQ ID NO: 226 - protein, 12 aa, Artificial Sequence
  Amino acid Sequence of aMTD895
AIIIVVPAIAAP

SEQ ID NO: 227 - protein, 12 aa, Artificial Sequence
  Amino acid Sequence of aMTD896
AILIVVAPIAAP

SEQ ID NO: 228 - protein, 12 aa, Artificial Sequence
  Amino acid Sequence of aMTD897
AVIVPVAIIAAP

SEQ ID NO: 229 - protein, 12 aa, Artificial Sequence
  Amino acid Sequence of aMTD899
AVVIALPAVVAP

SEQ ID NO: 230 - protein, 12 aa, Artificial Sequence
  Amino acid Sequence of aMTD900
ALVAVIAPVVAP

SEQ ID NO: 231 - protein, 12 aa, Artificial Sequence
  Amino acid Sequence of aMTD901
ALVAVLPAVAVP

SEQ ID NO: 232 - protein, 12 aa, Artificial Sequence
  Amino acid Sequence of aMTD902
ALVAPLLAVAVP

SEQ ID NO: 233 - protein, 12 aa, Artificial Sequence
  Amino acid Sequence of aMTD904
AVLAVVAPVVAP

SEQ ID NO: 234 - protein, 12 aa, Artificial Sequence
  Amino acid Sequence of aMTD905
AVIAVAPLVVAP

SEQ ID NO: 235 - protein, 12 aa, Artificial Sequence
  Amino acid Sequence of aMTD906
AVIALAPVVVAP

SEQ ID NO: 236 - protein, 12 aa, Artificial Sequence
  Amino acid Sequence of aMTD907
VAIALAPVVVAP

SEQ ID NO: 237 - protein, 12 aa, Artificial Sequence
  Amino acid Sequence of aMTD908
VALALAPVVVAP

SEQ ID NO: 238 - protein, 12 aa, Artificial Sequence
  Amino acid Sequence of aMTD910
VAALLPAVVVAP

SEQ ID NO: 239 - protein, 12 aa, Artificial Sequence
  Amino acid Sequence of aMTD911
VALALPAVVVAP

SEQ ID NO: 240 - protein, 12 aa, Artificial Sequence
  Amino acid Sequence of aMTD912
VALLAPAVVVAP

SEQ ID NO: 241 - DNA, 36 bp, Artificial Sequence
  cDNA Sequence of aMTD1
gcggcggcgctggcgccggtggtgctggcgctgccg

SEQ ID NO: 242 - DNA, 36 bp, Artificial Sequence
  cDNA Sequence of aMTD2
gcggcggcggtgccgctgctggcggtggtggtgccg

SEQ ID NO: 243 - DNA, 36 bp, Artificial Sequence
  cDNA Sequence of aMTD3
gcggcgctgctggtgccggcggcggtgctggcgccg

SEQ ID NO: 244 - DNA, 36 bp, Artificial Sequence
  cDNA Sequence of aMTD4
gcgctggcgctgctgccggtggcggcgctggcgccg

SEQ ID NO: 245 - DNA, 36 bp, Artificial Sequence
  cDNA Sequence of aMTD5
gcggcggcgctgctgccggtggcgctggtggcgccg

SEQ ID NO: 246 - DNA, 36 bp, Artificial Sequence
  cDNA Sequence of aMTD11
gtggtggcgctggcgccggcgctggcggcgctgccg

SEQ ID NO: 247 - DNA, 36 bp, Artificial Sequence
  cDNA Sequence of aMTD12
ctgctggcggcggtgccggcggtgctgctggcgccg

SEQ ID NO: 248 - DNA, 36 bp, Artificial Sequence
  cDNA Sequence of aMTD13
gcggcggcgctggtgccggtggtggcgctgctgccg

SEQ ID NO: 249 - DNA, 36 bp, Artificial Sequence
  cDNA Sequence of aMTD21
gcggtggcgctgctgccggcgctgctggcggtgccg

SEQ ID NO: 250 - DNA, 36 bp, Artificial Sequence
  cDNA Sequence of aMTD22
gcggtggtgctggtgccggtgctggcggcggcgccg

SEQ ID NO: 251 - DNA, 36 bp, Artificial Sequence
  cDNA Sequence of aMTD23
gtggtgctggtgctgccggcggcggcggcggtgccg

SEQ ID NO: 252 - DNA, 36 bp, Artificial Sequence
  cDNA Sequence of aMTD24
attgcgctggcggcgccggcgctgattgtggcgccg

SEQ ID NO: 253 - DNA, 36 bp, Artificial Sequence
  cDNA Sequence of aMTD25
attgtggcggtggcgccggcgctggtggcgctgccg

SEQ ID NO: 254 - DNA, 36 bp, Artificial Sequence
  Polynucleotide Sequence of aMTD42
gtggcggcgctgccggtggtggcggtggtggcgccg

SEQ ID NO: 255 - DNA, 36 bp, Artificial Sequence
  cDNA Sequence of aMTD43
ctgctggcggcgccgctggtggtggcggcggtgccg

SEQ ID NO: 256 - DNA, 36 bp, Artificial Sequence
  cDNA Sequence of aMTD44
gcgctggcggtgccggtggcgctgctggtggcgccg

SEQ ID NO: 257 - DNA, 36 bp, Artificial Sequence
  cDNA Sequence of aMTD61
gtggcggcgctgccggtgctgctggcggcgctgccg

SEQ ID NO: 258 - DNA, 36 bp, Artificial Sequence
  cDNA Sequence of aMTD62
gtggcgctgctggcgccggtggcgctggcggtgccg

SEQ ID NO: 259 - DNA, 36 bp, Artificial Sequence
  cDNA Sequence of aMTD63
gcggcgctgctggtgccggcgctggtggcggtgccg

SEQ ID NO: 260 - DNA, 36 bp, Artificial Sequence
  cDNA Sequence of aMTD64
gcgattgtggcgctgccggtggcggtgctggcgccg

SEQ ID NO: 261 - DNA, 36 bp, Artificial Sequence
  cDNA Sequence of aMTD65
attgcgattgtggcgccggtggtggcgctggcgccg

SEQ ID NO: 262 - DNA, 36 bp, Artificial Sequence
  cDNA Sequence of aMTD81
gcggcgctgctgccggcgctggcggcgctgctgccg

SEQ ID NO: 263 - DNA, 36 bp, Artificial Sequence
  cDNA Sequence of aMTD82
gcggtggtgctggcgccggtggcggcggtgctgccg

SEQ ID NO: 264 - DNA, 36 bp, Artificial Sequence
  cDNA Sequence of aMTD83
ctggcggtggcggcgccgctggcgctggcgctgccg

SEQ ID NO: 265 - DNA, 36 bp, Artificial Sequence
  cDNA Sequence of aMTD84
gcggcggtggcggcgccgctgctgctggcgctgccg

SEQ ID NO: 266 - DNA, 36 bp, Artificial Sequence
  cDNA Sequence of aMTD85
ctgctggtgctgccggcggcggcgctggcggcgccg

SEQ ID NO: 267 - DNA, 36 bp, Artificial Sequence
  cDNA Sequence of aMTD101
ctggtggcggtggcgccggtggcggcggtgctgccg

SEQ ID NO: 268 - DNA, 36 bp, Artificial Sequence
  cDNA Sequence of aMTD102
ctggcgctggcgccggcggcgctggcgctgctgccg

SEQ ID NO: 269 - DNA, 36 bp, Artificial Sequence
  cDNA Sequence of aMTD103
gcgctgattgcggcgccgattctggcgctggcgccg

SEQ ID NO: 270 - DNA, 36 bp, Artificial Sequence
  cDNA Sequence of aMTD104
gcggtggtggcggcgccgctggtgctggcgctgccg

SEQ ID NO: 271 - DNA, 36 bp, Artificial Sequence
  cDNA Sequence of aMTD105
ctgctggcgctggcgccggcggcgctgctggcgccg

SEQ ID NO: 272 - DNA, 36 bp, Artificial Sequence
  cDNA Sequence of aMTD121
gcgattgtggcgctgccggcgctggcgctggcgccg

SEQ ID NO: 273 - DNA, 36 bp, Artificial Sequence
  cDNA Sequence of aMTD123
gcggcgattattgtgccggcggcgctgctggcgccg

SEQ ID NO: 274 - DNA, 36 bp, Artificial Sequence
  cDNA Sequence of aMTD124
attgcggtggcgctgccggcgctgattgcggcgccg

SEQ ID NO: 275 - DNA, 36 bp, Artificial Sequence
  Polynucleotide Sequence of aMTD141
gcggtgattgtgctgccggcgctggcggtggcgccg

SEQ ID NO: 276 - DNA, 36 bp, Artificial Sequence
  Polynucleotide Sequence of aMTD143
gcggtgctggcggtgccggcggtgctggtggcgccg

SEQ ID NO: 277 - DNA, 36 bp, Artificial Sequence
  Polynucleotide Sequence of aMTD144
gtgctggcgattgtgccggcggtggcgctggcgccg

SEQ ID NO: 278 - DNA, 36 bp, Artificial Sequence
  Polynucleotide Sequence of aMTD145
ctgctggcggtggtgccggcggtggcgctggcgccg

SEQ ID NO: 279 - DNA, 36 bp, Artificial Sequence
  cDNA Sequence of aMTD161
gcggtgattgcgctgccggcgctgattgcggcgccg

SEQ ID NO: 280 - DNA, 36 bp, Artificial Sequence
  cDNA Sequence of aMTD162
gcggtggtggcgctgccggcggcgctgattgtgccg

SEQ ID NO: 281 - DNA, 36 bp, Artificial Sequence
  cDNA Sequence of aMTD163
ctggcgctggtgctgccggcggcgctggcggcgccg

SEQ ID NO: 282 - DNA, 36 bp, Artificial Sequence
  cDNA Sequence of aMTD164
ctggcggcggtgctgccggcgctgctggcggcgccg

SEQ ID NO: 283 - DNA, 36 bp, Artificial Sequence
  cDNA Sequence of aMTD165
gcgctggcggtgccggtggcgctggcgattgtgccg

SEQ ID NO: 284 - DNA, 36 bp, Artificial Sequence
  cDNA Sequence of aMTD182
gcgctgattgcgccggtggtggcgctggtggcgccg

SEQ ID NO: 285 - DNA, 36 bp, Artificial Sequence
  cDNA Sequence of aMTD183
ctgctggcggcgccggtggtgattgcgctggcgccg

SEQ ID NO: 286 - DNA, 36 bp, Artificial Sequence
  cDNA Sequence of aMTD184
ctggcggcgattgtgccggcgattattgcggtgccg

SEQ ID NO: 287 - DNA, 36 bp, Artificial Sequence
  cDNA Sequence of aMTD185
gcggcgctggtgctgccgctgattattgcggcgccg

SEQ ID NO: 288 - DNA, 36 bp, Artificial Sequence
  cDNA Sequence of aMTD201
ctggcgctggcggtgccggcgctggcggcgctgccg

SEQ ID NO: 289 - DNA, 36 bp, Artificial Sequence
  cDNA Sequence of aMTD204
ctgattgcggcgctgccggcggtggcggcgctgccg

SEQ ID NO: 290 - DNA, 36 bp, Artificial Sequence
  cDNA Sequence of aMTD205
gcgctggcgctggtgccggcgattgcggcgctgccg

SEQ ID NO: 291 - DNA, 36 bp, Artificial Sequence
  cDNA Sequence of aMTD221
gcggcgattctggcgccgattgtggcgctggcgccg

SEQ ID NO: 292 - DNA, 36 bp, Artificial Sequence
  cDNA Sequence of aMTD222
gcgctgctgattgcgccggcggcggtgattgcgccg

SEQ ID NO: 293 - DNA, 36 bp, Artificial Sequence
  cDNA Sequence of aMTD223
gcgattctggcggtgccgattgcggtggtggcgccg

SEQ ID NO: 294 - DNA, 36 bp, Artificial Sequence
  cDNA Sequence of aMTD224
attctggcggcggtgccgattgcgctggcggcgccg

SEQ ID NO: 295 - DNA, 36 bp, Artificial Sequence
  cDNA Sequence of aMTD225
gtggcggcgctgctgccggcggcggcggtgctgccg

SEQ ID NO: 296 - DNA, 36 bp, Artificial Sequence
  cDNA Sequence of aMTD241
gcggcggcggtggtgccggtgctgctggtggcgccg

SEQ ID NO: 297 - DNA, 36 bp, Artificial Sequence
  cDNA Sequence of aMTD242
gcggcgctgctggtgccggcgctggtggcggcgccg

SEQ ID NO: 298 - DNA, 36 bp, Artificial Sequence
  cDNA Sequence of aMTD243
gcggcggtgctgctgccggtggcgctggcggcgccg

SEQ ID NO: 299 - DNA, 36 bp, Artificial Sequence
  cDNA Sequence of aMTD245
gcggcggcgctggcgccggtgctggcgctggtgccg

SEQ ID NO: 300 - DNA, 36 bp, Artificial Sequence
  cDNA Sequence of aMTD261
ctggtgctggtgccgctgctggcggcggcggcgccg

SEQ ID NO: 301 - DNA, 36 bp, Artificial Sequence
  cDNA Sequence of aMTD262
gcgctgattgcggtgccggcgattattgtggcgccg

SEQ ID NO: 302 - DNA, 36 bp, Artificial Sequence
  cDNA Sequence of aMTD263
gcgctggcggtgattccggcggcggcgattctgccg

SEQ ID NO: 303 - DNA, 36 bp, Artificial Sequence
  cDNA Sequence of aMTD264
ctggcggcggcgccggtggtgattgtgattgcgccg

SEQ ID NO: 304 - DNA, 36 bp, Artificial Sequence
  cDNA Sequence of aMTD265
gtgctggcgattgcgccgctgctggcggcggtgccg

SEQ ID NO: 305 - DNA, 36 bp, Artificial Sequence
  cDNA Sequence of aMTD281
gcgctgattgtgctgccggcggcggtggcggtgccg

SEQ ID NO: 306 - DNA, 36 bp, Artificial Sequence
  cDNA Sequence of aMTD282
gtgctggcggtggcgccggcgctgattgtggcgccg

SEQ ID NO: 307 - DNA, 36 bp, Artificial Sequence
  cDNA Sequence of aMTD283
gcggcgctgctggcgccggcgctgattgtggcgccg

SEQ ID NO: 308 - DNA, 36 bp, Artificial Sequence
  cDNA Sequence of aMTD284
gcgctgattgcgccggcggtggcgctgattgtgccg

SEQ ID NO: 309 - DNA, 36 bp, Artificial Sequence
  cDNA Sequence of aMTD285
gcgattgtgctgctgccggcggcggtggtggcgccg

SEQ ID NO: 310 - DNA, 36 bp, Artificial Sequence
  cDNA Sequence of aMTD301
gtgattgcggcgccggtgctggcggtgctggcgccg

SEQ ID NO: 311 - DNA, 36 bp, Artificial Sequence
  cDNA Sequence of aMTD302
ctggcgctggcgccggcgctggcgctgctggcgccg

SEQ ID NO: 312 - DNA, 36 bp, Artificial Sequence
  cDNA Sequence of aMTD304
gcgattattctggcgccgattgcggcgattgcgccg

SEQ ID NO: 313 - DNA, 36 bp, Artificial Sequence
  cDNA Sequence of aMTD305
attgcgctggcggcgccgattctgctggcggcgccg

SEQ ID NO: 314 - DNA, 36 bp, Artificial Sequence
  cDNA Sequence of aMTD321
attgtggcggtggcgctgccggcgctggcggtgccg

SEQ ID NO: 315 - DNA, 36 bp, Artificial Sequence
  cDNA Sequence of aMTD322
gtggtggcgattgtgctgccggcgctggcggcgccg

SEQ ID NO: 316 - DNA, 36 bp, Artificial Sequence
  cDNA Sequence of aMTD323
attgtggcggtggcgctgccggtggcgctggcgccg

SEQ ID NO: 317 - DNA, 36 bp, Artificial Sequence
  cDNA Sequence of aMTD324
attgtggcggtggcgctgccggcggcgctggtgccg

SEQ ID NO: 318 - DNA, 36 bp, Artificial Sequence
  cDNA Sequence of aMTD325
attgtggcggtggcgctgccggcggtggcgctgccg

SEQ ID NO: 319 - DNA, 36 bp, Artificial Sequence
  cDNA Sequence of aMTD341
attgtggcggtggcgctgccggcggtgctggcgccg

SEQ ID NO: 320 - DNA, 36 bp, Artificial Sequence
  cDNA Sequence of aMTD342
gtgattgtggcgctggcgccggcggtgctggcgccg

SEQ ID NO: 321 - DNA, 36 bp, Artificial Sequence
  cDNA Sequence of aMTD343
attgtggcggtggcgctgccggcgctggtggcgccg

SEQ ID NO: 322 - DNA, 36 bp, Artificial Sequence
  cDNA Sequence of aMTD345
gcgctgctgattgtggcgccggtggcggtggcgccg

SEQ ID NO: 323 - DNA, 36 bp, Artificial Sequence
  cDNA Sequence of aMTD361
gcggtggtgattgtggcgccggcggtgattgcgccg

SEQ ID NO: 324 - DNA, 36 bp, Artificial Sequence
  cDNA Sequence of aMTD363
gcggtgctggcggtggcgccggcgctgattgtgccg

SEQ ID NO: 325 - DNA, 36 bp, Artificial Sequence
  cDNA Sequence of aMTD364
ctggtggcggcggtggcgccggcgctgattgtgccg

SEQ ID NO: 326 - DNA, 36 bp, Artificial Sequence
  cDNA Sequence of aMTD365
gcggtgattgtggtggcgccggcgctgctggcgccg

SEQ ID NO: 327 - DNA, 36 bp, Artificial Sequence
  cDNA Sequence of aMTD381
gtggtggcgattgtgctgccggcggtggcggcgccg

SEQ ID NO: 328 - DNA, 36 bp, Artificial Sequence
  cDNA Sequence of aMTD382
gcggcggcgctggtgattccggcgattctggcgccg

SEQ ID NO: 329 - DNA, 36 bp, Artificial Sequence
  cDNA Sequence of aMTD383
gtgattgtggcgctggcgccggcgctgctggcgccg

SEQ ID NO: 330 - DNA, 36 bp, Artificial Sequence
  cDNA Sequence of aMTD384
gtgattgtggcgattgcgccggcgctgctggcgccg

SEQ ID NO: 331 - DNA, 36 bp, Artificial Sequence
  cDNA Sequence of aMTD385
attgtggcgattgcggtgccggcgctggtggcgccg

SEQ ID NO: 332 - DNA, 36 bp, Artificial Sequence
  cDNA Sequence of aMTD401
gcggcgctggcggtgattccggcggcgattctgccg

SEQ ID NO: 333 - DNA, 36 bp, Artificial Sequence
  Polynucleotide of aMTD402
gcgctggcggcggtgattccggcggcgattctgccg

SEQ ID NO: 334 - DNA, 36 bp, Artificial Sequence
  cDNA Sequence of aMTD403
gcggcggcgctggtgattccggcggcgattctgccg

SEQ ID NO: 335 - DNA, 36 bp, Artificial Sequence
  cDNA Sequence of aMTD404
ctggcggcggcggtgattccggcggcgattctgccg

SEQ ID NO: 336 - DNA, 36 bp, Artificial Sequence
  cDNA Sequence of aMTD405
ctggcggcggcggtgattccggtggcgattctgccg

SEQ ID NO: 337 - DNA, 36 bp, Artificial Sequence
  cDNA Sequence of aMTD421
gcggcgattctggcggcgccgctgattgcggtgccg

SEQ ID NO: 338 - DNA, 36 bp, Artificial Sequence
  cDNA Sequence of aMTD422
gtggtggcgattctggcgccgctgctggcggcgccg

SEQ ID NO: 339 - DNA, 36 bp, Artificial Sequence
  cDNA Sequence of aMTD424
gcggtggtggtggcggcgccggtgctggcgctgccg

SEQ ID NO: 340 - DNA, 36 bp, Artificial Sequence
  cDNA Sequence of aMTD425
gcggtggtggcgattgcgccggtgctggcgctgccg

SEQ ID NO: 341 - DNA, 36 bp, Artificial Sequence
  cDNA Sequence of aMTD442
gcgctggcggcgctggtgccggcggtgctggtgccg

SEQ ID NO: 342 - DNA, 36 bp, Artificial Sequence
  cDNA Sequence of aMTD443
gcgctggcggcgctggtgccggtggcgctggtgccg

SEQ ID NO: 343 - DNA, 36 bp, Artificial Sequence
  cDNA Sequence of aMTD444
ctggcggcggcgctggtgccggtggcgctggtgccg

SEQ ID NO: 344 - DNA, 36 bp, Artificial Sequence
  cDNA Sequence of aMTD445
gcgctggcggcgctggtgccggcgctggtggtgccg

SEQ ID NO: 345 - DNA, 36 bp, Artificial Sequence
  cDNA Sequence of aMTD461
attgcggcggtgattgtgccggcggtggcgctgccg

SEQ ID NO: 346 - DNA, 36 bp, Artificial Sequence
  cDNA Sequence of aMTD462
attgcggcggtgctggtgccggcggtggcgctgccg

SEQ ID NO: 347 - DNA, 36 bp, Artificial Sequence
  cDNA Sequence of aMTD463
gcggtggcgattctggtgccgctgctggcggcgccg

SEQ ID NO: 348 - DNA, 36 bp, Artificial Sequence
  cDNA Sequence of aMTD464
gcggtggtgattctggtgccgctggcggcggcgccg

SEQ ID NO: 349 - DNA, 36 bp, Artificial Sequence
  cDNA Sequence of aMTD465
attgcggcggtgattgtgccggtggcggcgctgccg

SEQ ID NO: 350 - DNA, 36 bp, Artificial Sequence
  cDNA Sequence of aMTD481
gcgattgcgattgcgattgtgccggtggcgctgccg

SEQ ID NO: 351 - DNA, 36 bp, Artificial Sequence
  cDNA Sequence of aMTD482
attctggcggtggcggcgattccggtggcggtgccg

SEQ ID NO: 352 - DNA, 36 bp, Artificial Sequence
  cDNA Sequence of aMTD483
attctggcggcggcgattattccggcggcgctgccg

SEQ ID NO: 353 - DNA, 36 bp, Artificial Sequence
  cDNA Sequence of aMTD484
ctggcggtggtgctggcggcgccggcgattgtgccg

SEQ ID NO: 354 - DNA, 36 bp, Artificial Sequence
  cDNA Sequence of aMTD485
gcgattctggcggcgattgtgccgctggcggtgccg

SEQ ID NO: 355 - DNA, 36 bp, Artificial Sequence
  cDNA Sequence of aMTD501
gtgattgtggcgctggcggtgccggcgctggcgccg

SEQ ID NO: 356 - DNA, 36 bp, Artificial Sequence
  cDNA Sequence of aMTD502
gcgattgtggcgctggcggtgccggtgctggcgccg

SEQ ID NO: 357 - DNA, 36 bp, Artificial Sequence
  cDNA Sequence of aMTD503
gcggcgattattattgtgctgccggcggcgctgccg

SEQ ID NO: 358 - DNA, 36 bp, Artificial Sequence
  cDNA Sequence of aMTD504
ctgattgtggcgctggcggtgccggcgctggcgccg

SEQ ID NO: 359 - DNA, 36 bp, Artificial Sequence
  cDNA Sequence of aMTD505
gcgattattattgtgattgcgccggcggcggcgccg

SEQ ID NO: 360 - DNA, 36 bp, Artificial Sequence
  cDNA Sequence of aMTD521
ctggcggcgctgattgtggtgccggcggtggcgccg

SEQ ID NO: 361 - DNA, 36 bp, Artificial Sequence
  cDNA Sequence of aMTD522
gcgctgctggtgattgcggtgccggcggtggcgccg

SEQ ID NO: 362 - DNA, 36 bp, Artificial Sequence
  cDNA Sequence of aMTD524
gcggtggcgctgattgtggtgccggcgctggcgccg

SEQ ID NO: 363 - DNA, 36 bp, Artificial Sequence
  cDNA Sequence of aMTD525
gcgctggcgattgtggtggcgccggtggcggtgccg

SEQ ID NO: 364 - DNA, 36 bp, Artificial Sequence
  cDNA Sequence of aMTD541
ctgctggcgctgattattgcgccggcggcggcgccg

SEQ ID NO: 365 - DNA, 36 bp, Artificial Sequence
  cDNA Sequence of aMTD542
gcgctggcgctgattattgtgccggcggtggcgccg

SEQ ID NO: 366 - DNA, 36 bp, Artificial Sequence
  cDNA Sequence of aMTD543
ctgctggcggcgctgattgcgccggcggcgctgccg

SEQ ID NO: 367 - DNA, 36 bp, Artificial Sequence
  cDNA Sequence of aMTD544
attgtggcgctgattgtggcgccggcggcggtgccg

SEQ ID NO: 368 - DNA, 36 bp, Artificial Sequence
  cDNA Sequence of aMTD545
gtggtgctggtgctggcggcgccggcggcggtgccg

SEQ ID NO: 369 - DNA, 36 bp, Artificial Sequence
  cDNA Sequence of aMTD561
gcggcggtggcgattgtgctgccggcggtggtgccg

SEQ ID NO: 370 - DNA, 36 bp, Artificial Sequence
  cDNA Sequence of aMTD562
gcgctgattgcggcgattgtgccggcgctggtgccg

SEQ ID NO: 371 - DNA, 36 bp, Artificial Sequence
  cDNA Sequence of aMTD563
gcgctggcggtgattgtggtgccggcgctggcgccg

SEQ ID NO: 372 - DNA, 36 bp, Artificial Sequence
  cDNA Sequence of aMTD564
gtggcgattgcgctgattgtgccggcgctggcgccg

SEQ ID NO: 373 - DNA, 36 bp, Artificial Sequence
  cDNA Sequence of aMTD565
gtggcgattgtgctggtggcgccggcggtggcgccg

SEQ ID NO: 374 - DNA, 36 bp, Artificial Sequence
  cDNA Sequence of aMTD582
gtggcggtggcgctgattgtgccggcgctggcgccg

SEQ ID NO: 375 - DNA, 36 bp, Artificial Sequence
  cDNA Sequence of aMTD583
gcggtgattctggcgctggcgccgattgtggcgccg

SEQ ID NO: 376 - DNA, 36 bp, Artificial Sequence
  cDNA Sequence of aMTD585
gcgctgattgtggcgattgcgccggcgctggtgccg

SEQ ID NO: 377 - DNA, 36 bp, Artificial Sequence
  cDNA Sequence of aMTD601
gcggcgattctgattgcggtgccgattgcggcgccg

SEQ ID NO: 378 - DNA, 36 bp, Artificial Sequence
  cDNA Sequence of aMTD602
gtgattgtggcgctggcggcgccggtgctggcgccg

SEQ ID NO: 379 - DNA, 36 bp, Artificial Sequence
  cDNA Sequence of aMTD603
gtgctggtggcgctggcggcgccggtgattgcgccg

SEQ ID NO: 380 - DNA, 36 bp, Artificial Sequence
  cDNA Sequence of aMTD604
gtggcgctgattgcggtggcgccggcggtggtgccg

SEQ ID NO: 381 - DNA, 36 bp, Artificial Sequence
  cDNA Sequence of aMTD605
gtgattgcggcggtgctggcgccggtggcggtgccg

SEQ ID NO: 382 - DNA, 36 bp, Artificial Sequence
  cDNA Sequence of aMTD622
gcgctgattgtgctggcggcgccggtggcggtgccg

SEQ ID NO: 383 - DNA, 36 bp, Artificial Sequence
  cDNA Sequence of aMTD623
gtggcggcggcgattgcgctgccggcgattgtgccg

SEQ ID NO: 384 - DNA, 36 bp, Artificial Sequence
  cDNA Sequence of aMTD625
attctggcggcggcggcggcgccgctgattgtgccg

SEQ ID NO: 385 - DNA, 36 bp, Artificial Sequence
  cDNA Sequence of aMTD643
ctggcgctggtgctggcggcgccggcgattgtgccg

SEQ ID NO: 386 - DNA, 36 bp, Artificial Sequence
  cDNA Sequence of aMTD645
gcgctggcggtggtggcgctgccggcgattgtgccg

SEQ ID NO: 387 - DNA, 36 bp, Artificial Sequence
  cDNA Sequence of aMTD661
gcggcgattctggcgccgattgtggcggcgctgccg

SEQ ID NO: 388 - DNA, 36 bp, Artificial Sequence
  cDNA Sequence of aMTD664
attctgattgcgattgcgattccggcggcggcgccg

SEQ ID NO: 389 - DNA, 36 bp, Artificial Sequence
  cDNA Sequence of aMTD665
ctggcgattgtgctggcggcgccggtggcggtgccg

SEQ ID NO: 390 - DNA, 36 bp, Artificial Sequence
  cDNA Sequence of aMTD666
gcggcgattgcgattattgcgccggcgattgtgccg

SEQ ID NO: 391 - DNA, 36 bp, Artificial Sequence
  cDNA Sequence of aMTD667
ctggcggtggcgattgtggcgccggcgctggtgccg

SEQ ID NO: 392 - DNA, 36 bp, Artificial Sequence
  cDNA Sequence of aMTD683
ctggcgattgtgctggcggcgccggcggtgctgccg

SEQ ID NO: 393 - DNA, 36 bp, Artificial Sequence
  cDNA Sequence of aMTD684
gcggcgattgtgctggcgctgccggcggtgctgccg

SEQ ID NO: 394 - DNA, 36 bp, Artificial Sequence
  cDNA Sequence of aMTD685
gcgctgctggtggcggtgctgccggcggcgctgccg

SEQ ID NO: 395 - DNA, 36 bp, Artificial Sequence
  cDNA Sequence of aMTD686
gcggcgctggtggcggtgctgccggtggcgctgccg

SEQ ID NO: 396 - DNA, 36 bp, Artificial Sequence
  cDNA Sequence of aMTD687
attgtggcggtggcgctggtgccggcgctggcgccg

SEQ ID NO: 397 - DNA, 36 bp, Artificial Sequence; identical to SEQ ID NO: 396
  cDNA Sequence of aMTD703

SEQ ID NO: 398 - DNA, 36 bp, Artificial Sequence
  cDNA Sequence of aMTD705
attgtggcggtggcgctgctgccggcgctggcgccg

SEQ ID NO: 399 - DNA, 36 bp, Artificial Sequence
  cDNA Sequence of aMTD706
attgtggcggtggcgctgctgccggcggtggcgccg

SEQ ID NO: 400 - DNA, 36 bp, Artificial Sequence
  cDNA Sequence of aMTD707
attgtggcgctggcggtgctgccggcggtggcgccg

SEQ ID NO: 401 - DNA, 36 bp, Artificial Sequence
  cDNA Sequence of aMTD724
gtggcggtgctggcggtgctgccggcgctggcgccg

SEQ ID NO: 402 - DNA, 36 bp, Artificial Sequence
  cDNA Sequence of aMTD725
attgcggtgctggcggtggcgccggcggtgctgccg

SEQ ID NO: 403 - DNA, 36 bp, Artificial Sequence
  cDNA Sequence of aMTD726
ctggcggtggcgattattgcgccggcggtggcgccg

SEQ ID NO: 404 - DNA, 36 bp, Artificial Sequence
  cDNA Sequence of aMTD727
gtggcgctggcgattgcgctgccggcggtgctgccg

SEQ ID NO: 405 - DNA, 36 bp, Artificial Sequence
  cDNA Sequence of aMTD743
gcgattgcgattgcgctggtgccggtggcgctgccg

SEQ ID NO: 406 - DNA, 36 bp, Artificial Sequence
  cDNA Sequence of aMTD744
gcggcggtggtgattgtggcgccggtggcgctgccg

SEQ ID NO: 407 - DNA, 36 bp, Artificial Sequence
  cDNA Sequence of aMTD746
gcggcgattctggcgattgtggcgccgctggcgccg

SEQ ID NO: 408 - DNA, 36 bp, Artificial Sequence
  cDNA Sequence of aMTD747
gtggcgctgctggcgattgcgccggcgctggcgccg

SEQ ID NO: 409 - DNA, 36 bp, Artificial Sequence
  cDNA Sequence of aMTD763
gtggcggtgctgattgcggtgccggcgctggcgccg

SEQ ID NO: 410 - DNA, 36 bp, Artificial Sequence
  cDNA Sequence of aMTD764
gcggtggcgctggcggtgctgccggcggtggtgccg

SEQ ID NO: 411 - DNA, 36 bp, Artificial Sequence
  cDNA Sequence of aMTD765
gcggtggcgctggcggtggtgccggcggtgctgccg

SEQ ID NO: 412 - DNA, 36 bp, Artificial Sequence
  cDNA Sequence of aMTD766
attgtggtgattgcggtggcgccggcggtggcgccg

SEQ ID NO: 413 - DNA, 36 bp, Artificial Sequence
  cDNA Sequence of aMTD767
attgtggtggcggcggtggtgccggcgctggcgccg

SEQ ID NO: 414 - DNA, 36 bp, Artificial Sequence
  cDNA Sequence of aMTD783
attgtggcgctggtgccggcggtggcgattgcgccg

SEQ ID NO: 415 - DNA, 36 bp, Artificial Sequence
  cDNA Sequence of aMTD784
gtggcggcgctgccggcggtggcgctggtggtgccg

SEQ ID NO: 416 - DNA, 36 bp, Artificial Sequence
  cDNA Sequence of aMTD786
ctggtggcgattgcgccgctggcggtgctggcgccg

SEQ ID NO: 417 - DNA, 36 bp, Artificial Sequence
  cDNA Sequence of aMTD787
gcggtggcgctggtgccggtgattgtggcggcgccg

SEQ ID NO: 418 - DNA, 36 bp, Artificial Sequence
  cDNA Sequence of aMTD788
gcgattgcggtggcgattgcgccggtggcgctgccg

SEQ ID NO: 419 - DNA, 36 bp, Artificial Sequence
  cDNA Sequence of aMTD803
gcgattgcgctggcggtgccggtgctggcgctgccg

SEQ ID NO: 420 - DNA, 36 bp, Artificial Sequence
  cDNA Sequence of aMTD805
ctggtgctgattgcggcggcgccgattgcgctgccg

SEQ ID NO: 421 - DNA, 36 bp, Artificial Sequence
  cDNA Sequence of aMTD806
ctggtggcgctggcggtgccggcggcggtgctgccg

SEQ ID NO: 422 - DNA, 36 bp, Artificial Sequence
  cDNA Sequence of aMTD807
gcggtggcgctggcggtgccggcgctggtgctgccg

SEQ ID NO: 423 - DNA, 36 bp, Artificial Sequence
  cDNA Sequence of aMTD808
ctggtggtgctggcggcggcgccgctggcggtgccg

SEQ ID NO: 424 - DNA, 36 bp, Artificial Sequence
  cDNA Sequence of aMTD809
ctgattgtgctggcggcgccggcgctggcggcgccg

SEQ ID NO: 425 - DNA, 36 bp, Artificial Sequence
  cDNA Sequence of aMTD810
gtgattgtgctggcggcgccggcgctggcggcgccg

SEQ ID NO: 426 - DNA, 36 bp, Artificial Sequence
  cDNA Sequence of aMTD811
gcggtggtgctggcggtgccggcgctggcggtgccg

SEQ ID NO: 427 - DNA, 36 bp, Artificial Sequence
  cDNA Sequence of aMTD824
ctgattattgtggcggcggcgccggcggtggcgccg

SEQ ID NO: 428 - DNA, 36 bp, Artificial Sequence
  cDNA Sequence of aMTD825
attgtggcggtgattgtggcgccggcggtggcgccg

SEQ ID NO: 429 - DNA, 36 bp, Artificial Sequence
  cDNA Sequence of aMTD826
ctggtggcgctggcggcgccgattattgcggtgccg

SEQ ID NO: 430 - DNA, 36 bp, Artificial Sequence
  cDNA Sequence of aMTD827
attgcggcggtgctggcggcgccggcgctggtgccg

SEQ ID NO: 431 - DNA, 36 bp, Artificial Sequence
  cDNA Sequence of aMTD828
attgcgctgctggcggcgccgattattgcggtgccg

SEQ ID NO: 432 - DNA, 36 bp, Artificial Sequence
  cDNA Sequence of aMTD829
gcggcgctggcgctggtggcgccggtgattgtgccg

SEQ ID NO: 433 - DNA, 36 bp, Artificial Sequence
  cDNA Sequence of aMTD830
attgcgctggtggcggcgccggtggcgctggtgccg

SEQ ID NO: 434 - DNA, 36 bp, Artificial Sequence
  cDNA Sequence of aMTD831
attattgtggcggtggcgccggcggcgattgtgccg

SEQ ID NO: 435 - DNA, 36 bp, Artificial Sequence
  cDNA Sequence of aMTD832
gcggtggcggcgattgtgccggtgattgtggcgccg

SEQ ID NO: 436 - DNA, 36 bp, Artificial Sequence
  cDNA Sequence of aMTD843
gcggtgctggtgctggtggcgccggcggcggcgccg

SEQ ID NO: 437 - DNA, 36 bp, Artificial Sequence
  cDNA Sequence of aMTD844
gtggtggcgctgctggcgccgctgattgcggcgccg

SEQ ID NO: 438 - DNA, 36 bp, Artificial Sequence
  cDNA Sequence of aMTD845
gcggcggtggtgattgcgccgctgctggcggtgccg

SEQ ID NO: 439 - DNA, 36 bp, Artificial Sequence
  cDNA Sequence of aMTD846
attgcggtggcggtggcggcgccgctgctggtgccg

SEQ ID NO: 440 - DNA, 36 bp, Artificial Sequence
  cDNA Sequence of aMTD847
ctggtggcgattgtggtgctgccggcggtggcgccg

SEQ ID NO: 441 - DNA, 36 bp, Artificial Sequence
  cDNA Sequence of aMTD848
gcggtggcgattgtggtgctgccggcggtggcgccg

SEQ ID NO: 442 - DNA, 36 bp, Artificial Sequence
  cDNA Sequence of aMTD849
gcggtgattctgctggcgccgctgattgcggcgccg

SEQ ID NO: 443 - DNA, 36 bp, Artificial Sequence
  cDNA Sequence of aMTD850
ctggtgattgcgctggcggcgccggtggcgctgccg

SEQ ID NO: 444 - DNA, 36 bp, Artificial Sequence
  cDNA Sequence of aMTD851
gtgctggcggtggtgctgccggcggtggcgctgccg

SEQ ID NO: 445 - DNA, 36 bp, Artificial Sequence
  cDNA Sequence of aMTD852
gtgctggcggtggcggcgccggcggtgctgctgccg

SEQ ID NO: 446 - DNA, 36 bp, Artificial Sequence
  cDNA Sequence of aMTD863
gcggcggtggtgctgctgccgattattgcggcgccg

SEQ ID NO: 447 - DNA, 36 bp, Artificial Sequence
  cDNA Sequence of aMTD864
gcgctgctggtgattgcgccggcgattgcggtgccg

SEQ ID NO: 448 - DNA, 36 bp, Artificial Sequence
  cDNA Sequence of aMTD865
gcggtgctggtgattgcggtgccggcgattgcgccg

SEQ ID NO: 449 - DNA, 36 bp, Artificial Sequence
  cDNA Sequence of aMTD867
gcgctgctggtggtgattgcgccgctggcggcgccg

SEQ ID NO: 450 - DNA, 36 bp, Artificial Sequence
  cDNA Sequence of aMTD868
gtgctggtggcggcgattctgccggcggcgattccg

SEQ ID NO: 451 - DNA, 36 bp, Artificial Sequence
  cDNA Sequence of aMTD870
gtgctggtggcggcggtgctgccgattgcggcgccg

SEQ ID NO: 452 - DNA, 36 bp, Artificial Sequence
  cDNA Sequence of aMTD872
gtgctggcggcggcggtgctgccgctggtggtgccg

SEQ ID NO: 453 - DNA, 36 bp, Artificial Sequence
  cDNA Sequence of aMTD875
gcgattgcgattgtggtgccggcggtggcggtgccg

SEQ ID NO: 454 - DNA, 36 bp, Artificial Sequence
  cDNA Sequence of aMTD877
gtggcgattattgcggtgccggcggtggtggcgccg

SEQ ID NO: 455 - DNA, 36 bp, Artificial Sequence
  cDNA Sequence of aMTD878
attgtggcgctggtggcgccggcggcggtggtgccg

SEQ ID NO: 456 - DNA, 36 bp, Artificial Sequence
  cDNA Sequence of aMTD879
gcggcgattgtgctgctgccggcggtggtggtgccg

SEQ ID NO: 457 - DNA, 36 bp, Artificial Sequence
  cDNA Sequence of aMTD881
gcggcgctgattgtggtgccggcggtggcggtgccg

SEQ ID NO: 458 - DNA, 36 bp, Artificial Sequence
  cDNA Sequence of aMTD882
gcgattgcgctggtggtgccggcggtggcggtgccg

SEQ ID NO: 459 - DNA, 36 bp, Artificial Sequence
  cDNA Sequence of aMTD883
ctggcgattgtgccggcggcgattgcggcgctgccg

SEQ ID NO: 460 - DNA, 36 bp, Artificial Sequence
  cDNA Sequence of aMTD885
ctggtggcgattgcgccggcggtggcggtgctgccg

SEQ ID NO: 461 - DNA, 36 bp, Artificial Sequence
  cDNA Sequence of aMTD887
gtgctggcggtggcgccggcggtggcggtgctgccg

SEQ ID NO: 462 - DNA, 36 bp, Artificial Sequence
  cDNA Sequence of aMTD888
attctggcggtggtggcgattccggcggcggcgccg

SEQ ID NO: 463 - DNA, 36 bp, Artificial Sequence
  cDNA Sequence of aMTD889
attctggtggcggcggcgccgattgcggcgctgccg

SEQ ID NO: 464 - DNA, 36 bp, Artificial Sequence
  cDNA Sequence of aMTD891
attctggcggtggcggcgattccggcggcgctgccg

SEQ ID NO: 465 - DNA, 36 bp, Artificial Sequence
  cDNA Sequence of aMTD893
gtgattgcgattccggcgattctggcggcggcgccg

SEQ ID NO: 466 - DNA, 36 bp, Artificial Sequence
  cDNA Sequence of aMTD895
gcgattattattgtggtgccggcgattgcggcgccg

SEQ ID NO: 467 - DNA, 36 bp, Artificial Sequence
  cDNA Sequence of aMTD896
gcgattctgattgtggtggcgccgattgcggcgccg

SEQ ID NO: 468 - DNA, 36 bp, Artificial Sequence
  cDNA Sequence of aMTD897
gcggtgattgtgccggtggcgattattgcggcgccg

SEQ ID NO: 469 - DNA, 36 bp, Artificial Sequence
  cDNA Sequence of aMTD899
gcggtggtgattgcgctgccggcggtggtggcgccg

SEQ ID NO: 470 - DNA, 36 bp, Artificial Sequence
  cDNA Sequence of aMTD900
gcgctggtggcggtgattgcgccggtggtggcgccg

SEQ ID NO: 471 - DNA, 36 bp, Artificial Sequence
  cDNA Sequence of aMTD901
gcgctggtggcggtgctgccggcggtggcggtgccg

SEQ ID NO: 472 - DNA, 36 bp, Artificial Sequence
  cDNA Sequence of aMTD902
gcgctggtggcgccgctgctggcggtggcggtgccg

SEQ ID NO: 473 - DNA, 36 bp, Artificial Sequence
  cDNA Sequence of aMTD904
gcggtgctggcggtggtggcgccggtggtggcgccg

SEQ ID NO: 474 - DNA, 36 bp, Artificial Sequence
  cDNA Sequence of aMTD905
gcggtgattgcggtggcgccgctggtggtggcgccg

SEQ ID NO: 475 - DNA, 36 bp, Artificial Sequence
  cDNA Sequence of aMTD906
gcggtgattgcgctggcgccggtggtggtggcgccg

SEQ ID NO: 476 - DNA, 36 bp, Artificial Sequence
  cDNA Sequence of aMTD907
gtggcgattgcgctggcgccggtggtggtggcgccg

SEQ ID NO: 477 - DNA, 36 bp, Artificial Sequence
  cDNA Sequence of aMTD908
gtggcgctggcgctggcgccggtggtggtggcgccg

SEQ ID NO: 478 - DNA, 36 bp, Artificial Sequence
  cDNA Sequence of aMTD910
gtggcggcgctgctgccggcggtggtggtggcgccg

SEQ ID NO: 479 - DNA, 36 bp, Artificial Sequence
  cDNA Sequence of aMTD911
gtggcgctggcgctgccggcggtggtggtggcgccg

SEQ ID NO: 480 - DNA, 36 bp, Artificial Sequence
  cDNA Sequence of aMTD912
gtggcgctgctggcgccggcggtggtggtggcgccg

SEQ ID NO: 481 - DNA, 69 bp, Artificial Sequence
  cDNA Sequence of aMTD1 5'-primer
gggtttcatatggcggcggcgctggcgccggtggtgctggcgctgccggcaaatattaccgttttctat

SEQ ID NO: 482 - DNA, 69 bp, Artificial Sequence
  cDNA Sequence of aMTD2 5'-primer
gggtttcatatggcggcggcggtgccgctgctggcggtggtggtgccggcaaatattaccgttttctat

SEQ ID NO: 483 - DNA, 69 bp, Artificial Sequence
  cDNA Sequence of aMTD3 5'-primer
gggtttcatatggcggcgctgctggtgccggcggcggtgctggcgccggcaaatattaccgttttctat

SEQ ID NO: 484 - DNA, 69 bp, Artificial Sequence
  cDNA Sequence of aMTD4 5'-primer
gggtttcatatggcgctggcgctgctgccggtggcggcgctggcgccggcaaatattaccgttttctat

SEQ ID NO: 485 - DNA, 69 bp, Artificial Sequence
  cDNA Sequence of aMTD5 5'-primer
gggtttcatatggcggcggcgctgctgccggtggcgctggtggcgccggcaaatattaccgttttctat

SEQ ID NO: 486 - DNA, 69 bp, Artificial Sequence
  cDNA Sequence of aMTD6 5'-primer
gggtttcatatggtgattgcgatgattccggcggcgttttgggtggcggcaaatattaccgttttctat

SEQ ID NO: 487 - DNA, 69 bp, Artificial Sequence
  cDNA Sequence of aMTD9 5'-primer
gggtttcatatggtggcgctggtgccggcggcgctgattctgccgccggcaaatattaccgttttctat

SEQ ID NO: 488 - DNA, 69 bp, Artificial Sequence
  cDNA Sequence of aMTD11 5'-primer
gggtttcatatggtggtggcgctggcgccggcgctggcggcgctgccggcaaatattaccgttttctat

SEQ ID NO: 489 - DNA, 69 bp, Artificial Sequence
  cDNA Sequence of aMTD12 5'-primer
gggtttcatatgctgctggcggcggtgccggcggtgctgctggcgccggcaaatattaccgttttctat

SEQ ID NO: 490 - DNA, 69 bp, Artificial Sequence
  cDNA Sequence of aMTD13 5'-primer
gggtttcatatggcggcggcgctggtgccggtggtggcgctgctgccggcaaatattaccgttttctat

SEQ ID NO: 491 - DNA, 69 bp, Artificial Sequence
  cDNA Sequence of aMTD16 5'-primer
gggtttcatatgaacaacagctgcaccacctataccaacggcagccaggcaaatattaccgttttctat

SEQ ID NO: 492 - DNA, 69 bp, Artificial Sequence
  cDNA Sequence of aMTD17 5'-primer
gggtttcatatgggcggctgcagcgcgccgcagaccacctgcagcaacgcaaatattaccgttttctat

SEQ ID NO: 493 - DNA, 69 bp, Artificial Sequence
  cDNA Sequence of aMTD18 5'-primer
gggtttcatatgaactattgctgcaccccgaccaccaacggccagagcgcaaatattaccgttttctat

SEQ ID NO: 494 - DNA, 69 bp, Artificial Sequence
  cDNA Sequence of aMTD19 5'-primer
gggtttcatatgtatgtgagctgctgcacctataccaacggcagccaggcaaatattaccgttttctat

SEQ ID NO: 495 - DNA, 69 bp, Artificial Sequence
  cDNA Sequence of aMTD20 5'-primer
gggtttcatatgaactattgcaacacctgcccgacctatggccagagcgcaaatattaccgttttctat

SEQ ID NO: 496 - DNA, 69 bp, Artificial Sequence
  cDNA Sequence of aMTD21 5'-primer
gggtttcatatggcggtggcgctgctgccggcgctgctggcggtgccggcaaatattaccgttttctat

SEQ ID NO: 497 - DNA, 69 bp, Artificial Sequence
  cDNA Sequence of aMTD22 5'-primer
gggtttcatatggcggtggtgctggtgccggtgctggcggcggcgccggcaaatattaccgttttctat

SEQ ID NO: 498 - DNA, 69 bp, Artificial Sequence
  cDNA Sequence of aMTD23 5'-primer
gggtttcatatggtggtgctggtgctgccggcggcggcggcggtgccggcaaatattaccgttttctat

SEQ ID NO: 499 - DNA, 69 bp, Artificial Sequence
  cDNA Sequence of aMTD24 5'-primer
gggtttcatatgattgcgctggcggcgccggcgctgattgtggcgccggcaaatattaccgttttctat

SEQ ID NO: 500 - DNA, 69 bp, Artificial Sequence
  cDNA Sequence of aMTD25 5'-primer
gggtttcatatgattgtggcggtggcgccggcgctggtggcgctgccggcaaatattaccgttttctat

SEQ ID NO: 501 - DNA, 69 bp, Artificial Sequence
  cDNA Sequence of aMTD26 5'-primer
gggtttcatatggcggcgattgcgctggcggcgccgctggcgattgtggcaaatattaccgttttctat

SEQ ID NO: 502 - DNA, 69 bp, Artificial Sequence
  cDNA Sequence of aMTD27 5'-primer
gggtttcatatgctggcgattgtggcggcggcggcggcgctggtggcggcaaatattaccgttttctat

SEQ ID NO: 503 - DNA, 69 bp, Artificial Sequence
  cDNA Sequence of aMTD28 5'-primer
gggtttcatatggcggtgccgctgctgccgctggtgccggcggtgccggcaaatattaccgttttctat

SEQ ID NO: 504 - DNA, 69 bp, Artificial Sequence
  cDNA Sequence of aMTD29 5'-primer
gggtttcatatggtgctgccgccgctgccggtgctgccggtgctgccggcaaatattaccgttttctat

SEQ ID NO: 505 - DNA, 69 bp, Artificial Sequence
  cDNA Sequence of aMTD30 5'-primer
gggtttcatatggcgatggcgctgctgccggcggcggtggcggtggcggcaaatattaccgttttctat

SEQ ID NO: 506 - DNA, 69 bp, Artificial Sequence
  cDNA Sequence of aMTD33 5'-primer
gggtttcatatggcggcggcgattctggcgccggcgtttctggcggtggcaaatattaccgttttctat

SEQ ID NO: 507 - DNA, 69 bp, Artificial Sequence
  cDNA Sequence of aMTD37 5'-primer
gggtttcatatgtattataaccagagcacctgcggcggccagtgctatgcaaatattaccgttttctat

SEQ ID NO: 508 - DNA, 69 bp, Artificial Sequence
  cDNA Sequence of aMTD38 5'-primer
gggtttcatatgaccacctgcagccagcagcagtattgcaccaacggcgcaaatattaccgttttctat

SEQ ID NO: 509 - DNA, 69 bp, Artificial Sequence
  cDNA Sequence of aMTD39 5'-primer
gggtttcatatgtgctataacaccagcccgtgcaccggctgctgctatgcaaatattaccgttttctat

SEQ ID NO: 510 - DNA, 69 bp, Artificial Sequence
  cDNA Sequence of aMTD40 5'-primer
gggtttcatatgacctataacaccagctgcaccccgggcacctgctatgcaaatattaccgttttctat

SEQ ID NO: 511 - DNA, 69 bp, Artificial Sequence
  cDNA Sequence of aMTD42 5'-primer
gggtttcatatggtggcggcgctgccggtggtggcggtggtggcgccggcaaatattaccgttttctat

SEQ ID NO: 512 - DNA, 69 bp, Artificial Sequence
  cDNA Sequence of aMTD43 5'-primer
gggtttcatatgctgctggcggcgccgctggtggtggcggcggtgccggcaaatattaccgttttctat

SEQ ID NO: 513 - DNA, 69 bp, Artificial Sequence
  cDNA Sequence of aMTD44 5'-primer
gggtttcatatggcgctggcggtgccggtggcgctgctggtggcgccggcaaatattaccgttttctat

SEQ ID NO: 514 - DNA, 69 bp, Artificial Sequence
  cDNA Sequence of aMTD49 5'-primer
gggtttcatatggtggtgccggcggcgccggcggtgccggtggtgccggcaaatattaccgttttctat

SEQ ID NO: 515 - DNA, 69 bp, Artificial Sequence
  cDNA Sequence of aMTD54 5'-primer
gggtttcatatgctggcggtggcggcgccgccggtggtggcgctgctggcaaatattaccgttttctat

SEQ ID NO: 516 - DNA, 69 bp, Artificial Sequence
  cDNA Sequence of aMTD57 5'-primer
gggtttcatatgcagaacaactgcaacaccagcagccagggcggcggcgcaaatattaccgttttctat

SEQ ID NO: 517 - DNA, 69 bp, Artificial Sequence
  cDNA Sequence of aMTD59 5'-primer
gggtttcatatggcggtgctggcggcgccggtggtggcggcgctggcggcaaatattaccgttttctat

SEQ ID NO: 518 - DNA, 69 bp, Artificial Sequence
  cDNA Sequence of aMTD61 5'-primer
gggtttcatatggtggcggcgctgccggtgctgctggcggcgctgccggcaaatattaccgttttctat

SEQ ID NO: 519 - DNA, 69 bp, Artificial Sequence
  cDNA Sequence of aMTD62 5'-primer
gggtttcatatggtggcgctgctggcgccggtggcgctggcggtgccggcaaatattaccgttttctat

SEQ ID NO: 520 - DNA, 69 bp, Artificial Sequence
  cDNA Sequence of aMTD63 5'-primer
gggtttcatatggcggcgctgctggtgccggcgctggtggcggtgccggcaaatattaccgttttctat

SEQ ID NO: 521 - DNA, 69 bp, Artificial Sequence
  cDNA Sequence of aMTD64 5'-primer
gggtttcatatggcgattgtggcgctgccggtggcggtgctggcgccggcaaatattaccgttttctat

SEQ ID NO: 522 - DNA, 69 bp, Artificial Sequence
  cDNA Sequence of aMTD65 5'-primer
gggtttcatatgattgcgattgtggcgccggtggtggcgctggcgccggcaaatattaccgttttctat

SEQ ID NO: 523 - DNA, 69 bp, Artificial Sequence
  cDNA Sequence of aMTD66 5'-primer
gggtttcatatggcgggcgtgctgggcggcccgattatgggcgtgccggcaaatattaccgttttctat

SEQ ID NO: 524 - DNA, 69 bp, Artificial Sequence
  cDNA Sequence of aMTD67 5'-primer
gggtttcatatgctggatgcggaagtgccgctggcggatgatgtgccggcaaatattaccgttttctat

SEQ ID NO: 525 - DNA, 69 bp, Artificial Sequence
  cDNA Sequence of aMTD68 5'-primer
gggtttcatatggtggcgccggtgctgccggcggcgccgctggtgccggcaaatattaccgttttctat

SEQ ID NO: 526 - DNA, 69 bp, Artificial Sequence
  cDNA Sequence of aMTD69 5'-primer
gggtttcatatgccggtggcggtgctgccgccggcggcgctggtgccggcaaatattaccgttttctat

SEQ ID NO: 527 - DNA, 69 bp, Artificial Sequence
  cDNA Sequence of aMTD71 5'-primer
gggtttcatatgtttatgtggatgtggtttccgtttatgtggtatccggcaaatattaccgttttctat

SEQ ID NO: 528 - DNA, 69 bp, Artificial Sequence
  cDNA Sequence of aMTD77 5'-primer
gggtttcatatggcgatgctgctgatgccgattgtgctgattgcgccggcaaatattaccgttttctat

SEQ ID NO: 529 - DNA, 69 bp, Artificial Sequence
  cDNA Sequence of aMTD81 5'-primer
gggtttcatatggcggcgctgctgccggcgctggcggcgctgctgccggcaaatattaccgttttctat

SEQ ID NO: 530 - DNA, 69 bp, Artificial Sequence
  cDNA Sequence of aMTD82 5'-primer
gggtttcatatggcggtggtgctggcgccggtggcggcggtgctgccggcaaatattaccgttttctat

SEQ ID NO: 531 - DNA, 69 bp, Artificial Sequence
  cDNA Sequence of aMTD83 5'-primer
gggtttcatatgctggcggtggcggcgccgctggcgctggcgctgccggcaaatattaccgttttctat

SEQ ID NO: 532 - DNA, 69 bp, Artificial Sequence
  cDNA Sequence of aMTD84 5'-primer
gggtttcatatggcggcggtggcggcgccgctgctgctggcgctgccggcaaatattaccgttttctat

SEQ ID NO: 533 - DNA, 69 bp, Artificial Sequence
  cDNA Sequence of aMTD85 5'-primer
gggtttcatatgctgctggtgctgccggcggcggcgctggcggcgccggcaaatattaccgttttctat

SEQ ID NO: 534 - DNA, 69 bp, Artificial Sequence
  cDNA Sequence of aMTD97 5'-primer
gggtttcatatggcgctgctggcggcgccgccggcgctgctggcgctggcaaatattaccgttttctat

SEQ ID NO: 535 - DNA, 69 bp, Artificial Sequence
  cDNA Sequence of aMTD101 5'-primer
gggtttcatatgctggtggcggtggcgccggtggcggcggtgctgccggcaaatattaccgttttctat

SEQ ID NO: 536 - DNA, 69 bp, Artificial Sequence
  cDNA Sequence of aMTD102 5'-primer
gggtttcatatgctggcgctggcgccggcggcgctggcgctgctgccggcaaatattaccgttttctat

SEQ ID NO: 537 - DNA, 69 bp, Artificial Sequence
  cDNA Sequence of aMTD103 5'-primer
gggtttcatatggcgctgattgcggcgccgattctggcgctggcgccggcaaatattaccgttttctat

SEQ ID NO: 538 - DNA, 69 bp, Artificial Sequence
  cDNA Sequence of aMTD104 5'-primer
gggtttcatatggcggtggtggcggcgccgctggtgctggcgctgccggcaaatattaccgttttctat

SEQ ID NO: 539 - DNA, 69 bp, Artificial Sequence
  cDNA Sequence of aMTD105 5'-primer
gggtttcatatgctgctggcgctggcgccggcggcgctgctggcgccggcaaatattaccgttttctat

SEQ ID NO: 540 - DNA, 69 bp, Artificial Sequence
  cDNA Sequence of aMTD113 5'-primer
gggtttcatatgccggtggcggtggcgctgctgattgcggtgccgccggcaaatattaccgttttctat

SEQ ID NO: 541 - DNA, 69 bp, Artificial Sequence
  cDNA Sequence of aMTD121 5'-primer
gggtttcatatggcgattgtggcgctgccggcgctggcgctggcgccggcaaatattaccgttttctat

SEQ ID NO: 542 - DNA, 69 bp, Artificial Sequence
  cDNA Sequence of aMTD123 5'-primer
gggtttcatatggcggcgattattgtgccggcggcgctgctggcgccggcaaatattaccgttttctat

SEQ ID NO: 543 - DNA, 69 bp, Artificial Sequence
  cDNA Sequence of aMTD124 5'-primer
gggtttcatatgattgcggtggcgctgccggcgctgattgcggcgccggcaaatattaccgttttctat

SEQ ID NO: 544 - DNA, 69 bp, Artificial Sequence
  cDNA Sequence of aMTD131 5'-primer
gggtttcatatgtggattattgcgccggtgtggctggcgtggattgcggcaaatattaccgttttctat

SEQ ID NO: 545 - DNA, 69 bp, Artificial Sequence
  cDNA Sequence of aMTD138 5'-primer
gggtttcatatgccgccggcggcgctgctggcgattctggcggtggcggcaaatattaccgttttctat

SEQ ID NO: 546 - DNA, 69 bp, Artificial Sequence
  cDNA Sequence of aMTD139 5'-primer
gggtttcatatgaccggcagcaccaacagcccgacctgcaccagcaccgcaaatattaccgttttctat

SEQ ID NO: 547 - DNA, 69 bp, Artificial Sequence
  cDNA Sequence of aMTD141 5'-primer
gggtttcatatggcggtgattgtgctgccggcgctggcggtggcgccggcaaatattaccgttttctat

SEQ ID NO: 548 - DNA, 69 bp, Artificial Sequence
  cDNA Sequence of aMTD142 5'-primer
gggtttcatatgctgctggcggcggtgccggtggcgctggtggcgccggcaaatattaccgttttctat

SEQ ID NO: 549 - DNA, 69 bp, Artificial Sequence
  cDNA Sequence of aMTD143 5'-primer
gggtttcatatggcggtgctggcggtgccggcggtgctggtggcgccggcaaatattaccgttttctat

SEQ ID NO: 550 - DNA, 69 bp, Artificial Sequence; identical to SEQ ID NO: 549
  cDNA Sequence of aMTD144 5'-primer

SEQ ID NO: 551 - DNA, 69 bp, Artificial Sequence
  cDNA Sequence of aMTD145 5'-primer
gggtttcatatgctgctggcggtggtgccggcggtggcgctggcgccggcaaatattaccgttttctat

SEQ ID NO: 552 - DNA, 69 bp, Artificial Sequence
  cDNA Sequence of aMTD152 5'-primer
gggtttcatatgctggcggcggcggtggcggcggtggcggcgctgctggcaaatattaccgttttctat

SEQ ID NO: 553 - DNA, 69 bp, Artificial Sequence
  cDNA Sequence of aMTD159 5'-primer
gggtttcatatgtgctatagcggcagcaccagccagaaccagccgccggcaaatattaccgttttctat

SEQ ID NO: 554 - DNA, 69 bp, Artificial Sequence
  cDNA Sequence of aMTD161 5'-primer
gggtttcatatggcggtgattgcgctgccggcgctgattgcggcgccggcaaatattaccgttttctat

SEQ ID NO: 555 - DNA, 69 bp, Artificial Sequence
  cDNA Sequence of aMTD162 5'-primer
gggtttcatatggcggtggtggcgctgccggcggcgctgattgtgccggcaaatattaccgttttctat

SEQ ID NO: 556 - DNA, 69 bp, Artificial Sequence
  cDNA Sequence of aMTD163 5'-primer
gggtttcatatgctggcgctggtgctgccggcggcgctggcggcgccggcaaatattaccgttttctat

SEQ ID NO: 557 - DNA, 69 bp, Artificial Sequence
  cDNA Sequence of aMTD164 5'-primer
gggtttcatatgctggcggcggtgctgccggcgctgctggcggcgccggcaaatattaccgttttctat

SEQ ID NO: 558 - DNA, 69 bp, Artificial Sequence
  cDNA Sequence of aMTD165 5'-primer
gggtttcatatggcgctggcggtgccggtggcgctggcgattgtgccggcaaatattaccgttttctat

SEQ ID NO: 559 - DNA, 69 bp, Artificial Sequence
  cDNA Sequence of aMTD167 5'-primer
gggtttcatatggtggcgattgcgattccggcggcgctggcgattccggcaaatattaccgttttctat

SEQ ID NO: 560 - DNA, 69 bp, Artificial Sequence
  cDNA Sequence of aMTD169 5'-primer
gggtttcatatggtggcgctggtggcgccggcgctgattctggcgccggcaaatattaccgttttctat

SEQ ID NO: 561 - DNA, 69 bp, Artificial Sequence
  cDNA Sequence of aMTD182 5'-primer
gggtttcatatggcgctgattgcgccggtggtggcgctggtggcgccggcaaatattaccgttttctat

SEQ ID NO: 562 - DNA, 69 bp, Artificial Sequence
  cDNA Sequence of aMTD183 5'-primer
gggtttcatatgctgctggcggcgccggtggtgattgcgctggcgccggcaaatattaccgttttctat

SEQ ID NO: 563 - DNA, 69 bp, Artificial Sequence
  cDNA Sequence of aMTD184 5'-primer
gggtttcatatgctggcggcgattgtgccggcgattattgcggtgccggcaaatattaccgttttctat

SEQ ID NO: 564 - DNA, 69 bp, Artificial Sequence
  cDNA Sequence of aMTD185 5'-primer
gggtttcatatggcggcgctggtgctgccgctgattattgcggcgccggcaaatattaccgttttctat

SEQ ID NO: 565 - DNA, 69 bp, Artificial Sequence
  cDNA Sequence of aMTD189 5'-primer
gggtttcatatggtgattctggtggcgccggcggtgattgcgccgccggcaaatattaccgttttctat

SEQ ID NO: 566 - DNA, 69 bp, Artificial Sequence
  cDNA Sequence of aMTD190 5'-primer
gggtttcatatggcggcgattctggcgccggcggtgattgcgccgccggcaaatattaccgttttctat

SEQ ID NO: 567 - DNA, 69 bp, Artificial Sequence
  cDNA Sequence of aMTD201 5'-primer
gggtttcatatgctggcgctggcggtgccggcgctggcggcgctgccggcaaatattaccgttttctat

SEQ ID NO: 568 - DNA, 69 bp, Artificial Sequence
  cDNA Sequence of aMTD204 5'-primer
gggtttcatatgctgattgcggcgctgccggcggtggcggcgctgccggcaaatattaccgttttctat

SEQ ID NO: 569 - DNA, 69 bp, Artificial Sequence
  cDNA Sequence of aMTD205 5'-primer
gggtttcatatggcgctggcgctggtgccggcgattgcggcgctgccggcaaatattaccgttttctat

SEQ ID NO: 570 - DNA, 69 bp, Artificial Sequence
  cDNA Sequence of aMTD210 5'-primer
gggtttcatatggcgctgattgcgctgccggcgctgccggcgctgccggcaaatattaccgttttctat

SEQ ID NO: 571 - DNA, 69 bp, Artificial Sequence
  cDNA Sequence of aMTD214 5'-primer
gggtttcatatggcgctgattgtggcgccggcgctgatggcgctgccggcaaatattaccgttttctat

SEQ ID NO: 572 - DNA, 69 bp, Artificial Sequence
  cDNA Sequence of aMTD221 5'-primer
gggtttcatatggcggcgattctggcgccgattgtggcgctggcgccggcaaatattaccgttttctat

SEQ ID NO: 573 - DNA, 69 bp, Artificial Sequence
  cDNA Sequence of aMTD222 5'-primer
gggtttcatatggcgctgctgattgcgccggcggcggtgattgcgccggcaaatattaccgttttctat

SEQ ID NO: 574 - DNA, 69 bp, Artificial Sequence
  cDNA Sequence of aMTD223 5'-primer
gggtttcatatggcgattctggcggtgccgattgcggtggtggcgccggcaaatattaccgttttctat

SEQ ID NO: 575 - DNA, 69 bp, Artificial Sequence
  cDNA Sequence of aMTD224 5'-primer
gggtttcatatgattctggcggcggtgccgattgcgctggcggcgccggcaaatattaccgttttctat

SEQ ID NO: 576 - DNA, 69 bp, Artificial Sequence
  cDNA Sequence of aMTD225 5'-primer
gggtttcatatggtggcggcgctgctgccggcggcggcggtgctgccggcaaatattaccgttttctat

SEQ ID NO: 577 - DNA, 69 bp, Artificial Sequence
  cDNA Sequence of aMTD226 5'-primer
gggtttcatatggcgctggtggcggcgattccggcgctggcgattccggcaaatattaccgttttctat

SEQ ID NO: 578 - DNA, 69 bp, Artificial Sequence
  cDNA Sequence of aMTD227 5'-primer
gggtttcatatgctggcggcgattgtgccgattgcggcggcggtgccggcaaatattaccgttttctat

SEQ ID NO: 579 - DNA, 69 bp, Artificial Sequence
  cDNA Sequence of aMTD241 5'-primer
gggtttcatatggcggcggcggtggtgccggtgctgctggtggcgccggcaaatattaccgttttctat

SEQ ID NO: 580 - DNA, 69 bp, Artificial Sequence
  cDNA Sequence of aMTD242 5'-primer
gggtttcatatggcggcgctgctggtgccggcgctggtggcggcgccggcaaatattaccgttttctat

SEQ ID NO: 581 - DNA, 69 bp, Artificial Sequence
  cDNA Sequence of aMTD243 5'-primer
gggtttcatatggcggcggtgctgctgccggtggcgctggcggcgccggcaaatattaccgttttctat

SEQ ID NO: 582 - DNA, 69 bp, Artificial Sequence
  cDNA Sequence of aMTD245 5'-primer
gggtttcatatggcggcggcgctggcgccggtgctggcgctggtgccggcaaatattaccgttttctat

SEQ ID NO: 583 - DNA, 69 bp, Artificial Sequence
  cDNA Sequence of aMTD246 5'-primer
gggtttcatatggtggtggcggtgccgctgctggtggcgtttgcggcggcaaatattaccgttttctat

SEQ ID NO: 584 - DNA, 69 bp, Artificial Sequence
  cDNA Sequence of aMTD248 5'-primer
gggtttcatatggtggcggcgattgtgccgattgcggcgctggtgccggcaaatattaccgttttctat

SEQ ID NO: 585 - DNA, 69 bp, Artificial Sequence
  cDNA Sequence of aMTD261 5'-primer
gggtttcatatgctggtgctggtgccgctgctggcggcggcggcgccggcaaatattaccgttttctat

SEQ ID NO: 586 - DNA, 69 bp, Artificial Sequence
  cDNA Sequence of aMTD262 5'-primer
gggtttcatatggcgctgattgcggtgccggcgattattgtggcgccggcaaatattaccgttttctat

SEQ ID NO: 587 - DNA, 69 bp, Artificial Sequence
  cDNA Sequence of aMTD263 5'-primer
gggtttcatatggcgctggcggtgattccggcggcggcgattctgccggcaaatattaccgttttctat

SEQ ID NO: 588 - DNA, 69 bp, Artificial Sequence
  cDNA Sequence of aMTD264 5'-primer
gggtttcatatgctggcggcggcgccggtggtgattgtgattgcgccggcaaatattaccgttttctat

SEQ ID NO: 589 - DNA, 69 bp, Artificial Sequence
  cDNA Sequence of aMTD265 5'-primer
gggtttcatatggtgctggcgattgcgccgctgctggcggcggtgccggcaaatattaccgttttctat

SEQ ID NO: 590 - DNA, 69 bp, Artificial Sequence
  cDNA Sequence of aMTD281 5'-primer
gggtttcatatggcgctgattgtgctgccggcggcggtggcggtgccggcaaatattaccgttttctat

SEQ ID NO: 591 - DNA, 69 bp, Artificial Sequence
  cDNA Sequence of aMTD282 5'-primer
gggtttcatatggtgctggcggtggcgccggcgctgattgtggcgccggcaaatattaccgttttctat

SEQ ID NO: 592 - DNA, 69 bp, Artificial Sequence
  cDNA Sequence of aMTD283 5'-primer
gggtttcatatggcggcgctgctggcgccggcgctgattgtggcgccggcaaatattaccgttttctat

SEQ ID NO: 593 - DNA, 69 bp, Artificial Sequence
  cDNA Sequence of aMTD284 5'-primer
gggtttcatatggcgctgattgcgccggcggtggcgctgattgtgccggcaaatattaccgttttctat

SEQ ID NO: 594 - DNA, 69 bp, Artificial Sequence
  cDNA Sequence of aMTD285 5'-primer
gggtttcatatggcgattgtgctgctgccggcggcggtggtggcgccggcaaatattaccgttttctat

SEQ ID NO: 595 - DNA, 69 bp, Artificial Sequence
  cDNA Sequence of aMTD301 5'-primer
gggtttcatatggtgattgcggcgccggtgctggcggtgctggcgccggcaaatattaccgttttctat

SEQ ID NO: 596 - DNA, 69 bp, Artificial Sequence
  cDNA Sequence of aMTD302 5'-primer
gggtttcatatgctggcgctggcgccggcgctggcgctgctggcgccggcaaatattaccgttttctat

SEQ ID NO: 597 - DNA, 69 bp, Artificial Sequence
  cDNA Sequence of aMTD304 5'-primer
gggtttcatatggcgattattctggcgccgattgcggcgattgcgccggcaaatattaccgttttctat

SEQ ID NO: 598 - DNA, 69 bp, Artificial Sequence
  cDNA Sequence of aMTD305 5'-primer
gggtttcatatgattgcgctggcggcgccgattctgctggcggcgccggcaaatattaccgttttctat

SEQ ID NO: 599 - DNA, 69 bp, Artificial Sequence
  cDNA Sequence of aMTD321 5'-primer
gggtttcatatgattgtggcggtggcgctgccggcgctggcggtgccggcaaatattaccgttttctat

SEQ ID NO: 600 - DNA, 69 bp, Artificial Sequence
  cDNA Sequence of aMTD322 5'-primer
gggtttcatatggtggtggcgattgtgctgccggcgctggcggcgccggcaaatattaccgttttctat

SEQ ID NO: 601 - DNA, 69 bp, Artificial Sequence
  cDNA Sequence of aMTD323 5'-primer
gggtttcatatgattgtggcggtggcgctgccggtggcgctggcgccggcaaatattaccgttttctat

SEQ ID NO: 602 - DNA, 69 bp, Artificial Sequence
  cDNA Sequence of aMTD324 5'-primer
gggtttcatatgattgtggcggtggcgctgccggcggcgctggtgccggcaaatattaccgttttctat

SEQ ID NO: 603 - DNA, 69 bp, Artificial Sequence
  cDNA Sequence of aMTD325 5'-primer
gggtttcatatgattgtggcggtggcgctgccggcggtggcgctgccggcaaatattaccgttttctat

SEQ ID NO: 604 - DNA, 69 bp, Artificial Sequence
  cDNA Sequence of aMTD329 5'-primer
gggtttcatatgctgccggtgctggtgccggtggtgccggtggtgccggcaaatattaccgttttctat

SEQ ID NO: 605 - DNA, 69 bp, Artificial Sequence
  cDNA Sequence of aMTD331 5'-primer
gggtttcatatggtgccggtgctggtgccgctggtgccggtggtgccggcaaatattaccgttttctat

SEQ ID NO: 606 - DNA, 69 bp, Artificial Sequence
  cDNA Sequence of aMTD341 5'-primer
gggtttcatatgattgtggcggtggcgctgccggcggtgctggcgccggcaaatattaccgttttctat

SEQ ID NO: 607 - DNA, 69 bp, Artificial Sequence
  cDNA Sequence of aMTD342 5'-primer
gggtttcatatggtgattgtggcgctggcgccggcggtgctggcgccggcaaatattaccgttttctat

SEQ ID NO: 608 - DNA, 69 bp, Artificial Sequence
  cDNA Sequence of aMTD343 5'-primer
gggtttcatatgattgtggcggtggcgctgccggcgctggtggcgccggcaaatattaccgttttctat

SEQ ID NO: 609 - DNA, 69 bp, Artificial Sequence
  cDNA Sequence of aMTD345 5'-primer
gggtttcatatggcgctgctgattgtggcgccggtggcggtggcgccggcaaatattaccgttttctat

SEQ ID NO: 610 - DNA, 69 bp, Artificial Sequence
  cDNA Sequence of aMTD349 5'-primer
gggtttcatatggtgccggtgctggtgccggtggtgccggtggtgccggcaaatattaccgttttctat

SEQ ID NO: 611 - DNA, 69 bp, Artificial Sequence
  cDNA Sequence of aMTD350 5'-primer
gggtttcatatggtgccgattctggtgccggtggtgccggtggtgccggcaaatattaccgttttctat

SEQ ID NO: 612 - DNA, 69 bp, Artificial Sequence
  cDNA Sequence of aMTD361 5'-primer
gggtttcatatggcggtggtgattgtggcgccggcggtgattgcgccggcaaatattaccgttttctat

SEQ ID NO: 613 - DNA, 69 bp, Artificial Sequence
  cDNA Sequence of aMTD363 5'-primer
gggtttcatatggcggtgctggcggtggcgccggcgctgattgtgccggcaaatattaccgttttctat

SEQ ID NO: 614 - DNA, 69 bp, Artificial Sequence
  cDNA Sequence of aMTD364 5'-primer
gggtttcatatgctggtggcggcggtggcgccggcgctgattgtgccggcaaatattaccgttttctat

SEQ ID NO: 615 - DNA, 69 bp, Artificial Sequence
  cDNA Sequence of aMTD365 5'-primer
gggtttcatatggcggtgattgtggtggcgccggcgctgctggcgccggcaaatattaccgttttctat

SEQ ID NO: 616 - DNA, 69 bp, Artificial Sequence
  cDNA Sequence of aMTD381 5'-primer
gggtttcatatggtggtggcgattgtgctgccggcggtggcggcgccggcaaatattaccgttttctat

SEQ ID NO: 617 - DNA, 69 bp, Artificial Sequence
  cDNA Sequence of aMTD382 5'-primer
gggtttcatatggcggcggcgctggtgattccggcgattctggcgccggcaaatattaccgttttctat

SEQ ID NO: 618 - DNA, 69 bp, Artificial Sequence
  cDNA Sequence of aMTD383 5'-primer
gggtttcatatggtgattgtggcgctggcgccggcgctgctggcgccggcaaatattaccgttttctat

SEQ ID NO: 619 - DNA, 69 bp, Artificial Sequence
  cDNA Sequence of aMTD384 5'-primer
gggtttcatatggtgattgtggcgattgcgccggcgctgctggcgccggcaaatattaccgttttctat

SEQ ID NO: 620 - DNA, 69 bp, Artificial Sequence
  cDNA Sequence of aMTD385 5'-primer
gggtttcatatgattgtggcgattgcggtgccggcgctggtggcgccggcaaatattaccgttttctat

SEQ ID NO: 621 - DNA, 69 bp, Artificial Sequence
  cDNA Sequence of aMTD390 5'-primer
gggtttcatatggtgccgctgctggtgccggtggtgccggtggtgccggcaaatattaccgttttctat

SEQ ID NO: 622 - DNA, 69 bp, Artificial Sequence
  cDNA Sequence of aMTD401 5'-primer
gggtttcatatggcggcgctggcggtgattccggcggcgattctgccggcaaatattaccgttttctat

SEQ ID NO: 623 - DNA, 69 bp, Artificial Sequence
  cDNA Sequence of aMTD402 5'-primer
gggtttcatatggcgctggcggcggtgattccggcggcgattctgccggcaaatattaccgttttctat

SEQ ID NO: 624 - DNA, 69 bp, Artificial Sequence
  cDNA Sequence of aMTD403 5'-primer
gggtttcatatggcggcggcgctggtgattccggcggcgattctgccggcaaatattaccgttttctat

SEQ ID NO: 625 - DNA, 69 bp, Artificial Sequence
  cDNA Sequence of aMTD404 5'-primer
gggtttcatatgctggcggcggcggtgattccggcggcgattctgccggcaaatattaccgttttctat

SEQ ID NO: 626 - DNA, 69 bp, Artificial Sequence
  cDNA Sequence of aMTD405 5'-primer
gggtttcatatgctggcggcggcggtgattccggtggcgattctgccggcaaatattaccgttttctat

SEQ ID NO: 627 - DNA, 69 bp, Artificial Sequence
  cDNA Sequence of aMTD421 5'-primer
gggtttcatatggcggcgattctggcggcgccgctgattgcggtgccggcaaatattaccgttttctat

SEQ ID NO: 628 - DNA, 69 bp, Artificial Sequence
  cDNA Sequence of aMTD422 5'-primer
gggtttcatatggtggtggcgattctggcgccgctgctggcggcgccggcaaatattaccgttttctat

SEQ ID NO: 629 - DNA, 69 bp, Artificial Sequence
  cDNA Sequence of aMTD424 5'-primer
gggtttcatatggcggtggtggtggcggcgccggtgctggcgctgccggcaaatattaccgttttctat

SEQ ID NO: 630 - DNA, 69 bp, Artificial Sequence
  cDNA Sequence of aMTD425 5'-primer
gggtttcatatggcggtggtggcgattgcgccggtgctggcgctgccggcaaatattaccgttttctat

SEQ ID NO: 631 - DNA, 69 bp, Artificial Sequence
  cDNA Sequence of aMTD426 5'-primer
gggtttcatatggcggcggcgctggcgattccgctggcgattattccggcaaatattaccgttttctat

SEQ ID NO: 632 - DNA, 69 bp, Artificial Sequence
  cDNA Sequence of aMTD436 5'-primer
gggtttcatatggcggtggtgctggtgattatgccggcggcgattccggcaaatattaccgttttctat

SEQ ID NO: 633 - DNA, 69 bp, Artificial Sequence
  cDNA Sequence of aMTD442 5'-primer
gggtttcatatggcgctggcggcgctggtgccggcggtgctggtgccggcaaatattaccgttttctat

SEQ ID NO: 634 - DNA, 69 bp, Artificial Sequence
  cDNA Sequence of aMTD443 5'-primer
gggtttcatatggcgctggcggcgctggtgccggtggcgctggtgccggcaaatattaccgttttctat

SEQ ID NO: 635 - DNA, 69 bp, Artificial Sequence
  cDNA Sequence of aMTD444 5'-primer
gggtttcatatgctggcggcggcgctggtgccggtggcgctggtgccggcaaatattaccgttttctat

SEQ ID NO: 636 - DNA, 69 bp, Artificial Sequence
  cDNA Sequence of aMTD445 5'-primer
gggtttcatatggcgctggcggcgctggtgccggcgctggtggtgccggcaaatattaccgttttctat

SEQ ID NO: 637 - DNA, 69 bp, Artificial Sequence
  cDNA Sequence of aMTD461 5'-primer
gggtttcatatgattgcggcggtgattgtgccggcggtggcgctgccggcaaatattaccgttttctat

SEQ ID NO: 638 - DNA, 69 bp, Artificial Sequence
  cDNA Sequence of aMTD462 5'-primer
gggtttcatatgattgcggcggtgctggtgccggcggtggcgctgccggcaaatattaccgttttctat

SEQ ID NO: 639 - DNA, 69 bp, Artificial Sequence
  cDNA Sequence of aMTD463 5'-primer
gggtttcatatggcggtggcgattctggtgccgctgctggcggcgccggcaaatattaccgttttctat

SEQ ID NO: 640 - DNA, 69 bp, Artificial Sequence
  cDNA Sequence of aMTD464 5'-primer
gggtttcatatggcggtggtgattctggtgccgctggcggcggcgccggcaaatattaccgttttctat

SEQ ID NO: 641 - DNA, 69 bp, Artificial Sequence
  cDNA Sequence of aMTD465 5'-primer
gggtttcatatgattgcggcggtgattgtgccggtggcggcgctgccggcaaatattaccgttttctat

SEQ ID NO: 642 - DNA, 69 bp, Artificial Sequence
  cDNA Sequence of aMTD466 5'-primer
gggtttcatatgattattgcggcggcggcgccgctggcgattattccggcaaatattaccgttttctat

SEQ ID NO: 643 - DNA, 69 bp, Artificial Sequence
  cDNA Sequence of aMTD481 5'-primer
gggtttcatatggcgattgcgattgcgattgtgccggtggcgctgccggcaaatattaccgttttctat

SEQ ID NO: 644 - DNA, 69 bp, Artificial Sequence
  cDNA Sequence of aMTD482 5'-primer
gggtttcatatgattctggcggtggcggcgattccggtggcggtgccggcaaatattaccgttttctat

SEQ ID NO: 645 - DNA, 69 bp, Artificial Sequence
  cDNA Sequence of aMTD483 5'-primer
gggtttcatatgattctggcggcggcgattattccggcggcgctgccggcaaatattaccgttttctat

SEQ ID NO: 646 - DNA, 69 bp, Artificial Sequence
  cDNA Sequence of aMTD484 5'-primer
gggtttcatatgctggcggtggtgctggcggcgccggcgattgtgccggcaaatattaccgttttctat

SEQ ID NO: 647 - DNA, 69 bp, Artificial Sequence
  cDNA Sequence of aMTD485 5'-primer
gggtttcatatggcgattctggcggcgattgtgccgctggcggtgccggcaaatattaccgttttctat

SEQ ID NO: 648 - DNA, 69 bp, Artificial Sequence
  cDNA Sequence of aMTD501 5'-primer
gggtttcatatggtgattgtggcgctggcggtgccggcgctggcgccggcaaatattaccgttttctat

SEQ ID NO: 649 - DNA, 69 bp, Artificial Sequence
  cDNA Sequence of aMTD502 5'-primer
gggtttcatatggcgattgtggcgctggcggtgccggtgctggcgccggcaaatattaccgttttctat

SEQ ID NO: 650 - DNA, 69 bp, Artificial Sequence
  cDNA Sequence of aMTD503 5'-primer
gggtttcatatggcggcgattattattgtgctgccggcggcgctgccggcaaatattaccgttttctat

SEQ ID NO: 651 - DNA, 69 bp, Artificial Sequence
  cDNA Sequence of aMTD504 5'-primer
gggtttcatatgctgattgtggcgctggcggtgccggcgctggcgccggcaaatattaccgttttctat

SEQ ID NO: 652 - DNA, 69 bp, Artificial Sequence
  cDNA Sequence of aMTD505 5'-primer
gggtttcatatggcgattattattgtgattgcgccggcggcggcgccggcaaatattaccgttttctat

SEQ ID NO: 653 - DNA, 69 bp, Artificial Sequence
  cDNA Sequence of aMTD521 5'-primer
gggtttcatatgctggcggcgctgattgtggtgccggcggtggcgccggcaaatattaccgttttctat

SEQ ID NO: 654 - DNA, 69 bp, Artificial Sequence
  cDNA Sequence of aMTD522 5'-primer
gggtttcatatggcgctgctggtgattgcggtgccggcggtggcgccggcaaatattaccgttttctat

SEQ ID NO: 655 - DNA, 69 bp, Artificial Sequence
  cDNA Sequence of aMTD524 5'-primer
gggtttcatatggcggtggcgctgattgtggtgccggcgctggcgccggcaaatattaccgttttctat

SEQ ID NO: 656 - DNA, 69 bp, Artificial Sequence
  cDNA Sequence of aMTD525 5'-primer
gggtttcatatggcgctggcgattgtggtggcgccggtggcggtgccggcaaatattaccgttttctat

SEQ ID NO: 657 - DNA, 69 bp, Artificial Sequence
  cDNA Sequence of aMTD527 5'-primer
gggtttcatatgctggtgctggcggcggtggcgccgattgcgattccggcaaatattaccgttttctat

SEQ ID NO: 658 - DNA, 69 bp, Artificial Sequence
  cDNA Sequence of aMTD541 5'-primer
gggtttcatatgctgctggcgctgattattgcgccggcggcggcgccggcaaatattaccgttttctat

SEQ ID NO: 659 - DNA, 69 bp, Artificial Sequence
  cDNA Sequence of aMTD542 5'-primer
gggtttcatatggcgctggcgctgattattgtgccggcggtggcgccggcaaatattaccgttttctat

SEQ ID NO: 660 - DNA, 69 bp, Artificial Sequence
  cDNA Sequence of aMTD543 5'-primer
gggtttcatatgctgctggcggcgctgattgcgccggcggcgctgccggcaaatattaccgttttctat

SEQ ID NO: 661 - DNA, 69 bp, Artificial Sequence
  cDNA Sequence of aMTD544 5'-primer
gggtttcatatgattgtggcgctgattgtggcgccggcggcggtgccggcaaatattaccgttttctat

SEQ ID NO: 662 - DNA, 69 bp, Artificial Sequence
  cDNA Sequence of aMTD545 5'-primer
gggtttcatatggtggtgctggtgctggcggcgccggcggcggtgccggcaaatattaccgttttctat

SEQ ID NO: 663 - DNA, 69 bp, Artificial Sequence
  cDNA Sequence of aMTD561 5'-primer
gggtttcatatggcggcggtggcgattgtgctgccggcggtggtgccggcaaatattaccgttttctat

SEQ ID NO: 664 - DNA, 69 bp, Artificial Sequence
  cDNA Sequence of aMTD562 5'-primer
gggtttcatatggcgctgattgcggcgattgtgccggcgctggtgccggcaaatattaccgttttctat

SEQ ID NO: 665 - DNA, 69 bp, Artificial Sequence
  cDNA Sequence of aMTD563 5'-primer
gggtttcatatggcgctggcggtgattgtggtgccggcgctggcgccggcaaatattaccgttttctat

SEQ ID NO: 666 - DNA, 69 bp, Artificial Sequence
  cDNA Sequence of aMTD564 5'-primer
gggtttcatatggtggcgattgcgctgattgtgccggcgctggcgccggcaaatattaccgttttctat

SEQ ID NO: 667 - DNA, 69 bp, Artificial Sequence
  cDNA Sequence of aMTD565 5'-primer
gggtttcatatggtggcgattgtgctggtggcgccggcggtggcgccggcaaatattaccgttttctat

SEQ ID NO: 668 - DNA, 69 bp, Artificial Sequence
  cDNA Sequence of aMTD577 5'-primer
gggtttcatatggcggcggtgctgattgtgccgattatggtgatgccggcaaatattaccgttttctat

SEQ ID NO: 669 - DNA, 69 bp, Artificial Sequence
  cDNA Sequence of aMTD582 5'-primer
gggtttcatatggtggcggtggcgctgattgtgccggcgctggcgccggcaaatattaccgttttctat

SEQ ID NO: 670 - DNA, 69 bp, Artificial Sequence
  cDNA Sequence of aMTD583 5'-primer
gggtttcatatggcggtgattctggcgctggcgccgattgtggcgccggcaaatattaccgttttctat

SEQ ID NO: 671 - DNA, 69 bp, Artificial Sequence
  cDNA Sequence of aMTD585 5'-primer
gggtttcatatggcgctgattgtggcgattgcgccggcgctggtgccggcaaatattaccgttttctat

SEQ ID NO: 672 - DNA, 69 bp, Artificial Sequence
  cDNA Sequence of aMTD601 5'-primer
gggtttcatatggcggcgattctgattgcggtgccgattgcggcgccggcaaatattaccgttttctat

SEQ ID NO: 673 - DNA, 69 bp, Artificial Sequence
  cDNA Sequence of aMTD602 5'-primer
gggtttcatatggtgattgtggcgctggcggcgccggtgctggcgccggcaaatattaccgttttctat

SEQ ID NO: 674 - DNA, 69 bp, Artificial Sequence
  cDNA Sequence of aMTD603 5'-primer
gggtttcatatggtgctggtggcgctggcggcgccggtgattgcgccggcaaatattaccgttttctat

SEQ ID NO: 675 - DNA, 69 bp, Artificial Sequence
  cDNA Sequence of aMTD604 5'-primer
gggtttcatatggtggcgctgattgcggtggcgccggcggtggtgccggcaaatattaccgttttctat

SEQ ID NO: 676 - DNA, 69 bp, Artificial Sequence
  cDNA Sequence of aMTD605 5'-primer
gggtttcatatggtgattgcggcggtgctggcgccggtggcggtgccggcaaatattaccgttttctat

SEQ ID NO: 677 - DNA, 69 bp, Artificial Sequence
  cDNA Sequence of aMTD606 5'-primer
gggtttcatatggcggcggcgattgcggcgattccgattattattccggcaaatattaccgttttctat

SEQ ID NO: 678 - DNA, 69 bp, Artificial Sequence; identical to SEQ ID NO: 677
  cDNA Sequence of aMTD622 5'-primer

SEQ ID NO: 679 - DNA, 69 bp, Artificial Sequence
  cDNA Sequence of aMTD623 5'-primer
gggtttcatatggtggcggcggcgattgcgctgccggcgattgtgccggcaaatattaccgttttctat

SEQ ID NO: 680 - DNA, 69 bp, Artificial Sequence
  cDNA Sequence of aMTD625 5'-primer
gggtttcatatgattctggcggcggcggcggcgccgctgattgtgccggcaaatattaccgttttctat

SEQ ID NO: 681 - DNA, 69 bp, Artificial Sequence
  cDNA Sequence of aMTD635 5'-primer
gggtttcatatgggcagcaccggcggcagccagcagaacaaccagtatgcaaatattaccgttttctat

SEQ ID NO: 682 - DNA, 69 bp, Artificial Sequence
  cDNA Sequence of aMTD643 5'-primer
gggtttcatatgctggcgctggtgctggcggcgccggcgattgtgccggcaaatattaccgttttctat

SEQ ID NO: 683 - DNA, 69 bp, Artificial Sequence
  cDNA Sequence of aMTD645 5'-primer
gggtttcatatggcgctggcggtggtggcgctgccggcgattgtgccggcaaatattaccgttttctat

SEQ ID NO: 684 - DNA, 69 bp, Artificial Sequence
  cDNA Sequence of aMTD661 5'-primer
gggtttcatatggcggcgattctggcgccgattgtggcggcgctgccggcaaatattaccgttttctat

SEQ ID NO: 685 - DNA, 69 bp, Artificial Sequence
  cDNA Sequence of aMTD664 5'-primer
gggtttcatatgattctgattgcgattgcgattccggcggcggcgccggcaaatattaccgttttctat

SEQ ID NO: 686 - DNA, 69 bp, Artificial Sequence
  cDNA Sequence of aMTD665 5'-primer
gggtttcatatgctggcgattgtgctggcggcgccggtggcggtgccggcaaatattaccgttttctat

SEQ ID NO: 687 - DNA, 69 bp, Artificial Sequence
  cDNA Sequence of aMTD666 5'-primer
gggtttcatatggcggcgattgcgattattgcgccggcgattgtgccggcaaatattaccgttttctat

SEQ ID NO: 688 - DNA, 69 bp, Artificial Sequence
  cDNA Sequence of aMTD667 5'-primer
gggtttcatatgctggcggtggcgattgtggcgccggcgctggtgccggcaaatattaccgttttctat

SEQ ID NO: 689 - DNA, 69 bp, Artificial Sequence
  cDNA Sequence of aMTD676 5'-primer
gggtttcatatggtgccgctgctggtgccggtgccggtggtggtgccggcaaatattaccgttttctat

SEQ ID NO: 690 - DNA, 69 bp, Artificial Sequence
  cDNA Sequence of aMTD683 5'-primer
gggtttcatatgctggcgattgtgctggcggcgccggcggtgctgccggcaaatattaccgttttctat

SEQ ID NO: 691 - DNA, 69 bp, Artificial Sequence
  cDNA Sequence of aMTD684 5'-primer
gggtttcatatggcggcgattgtgctggcgctgccggcggtgctgccggcaaatattaccgttttctat

SEQ ID NO: 692 - DNA, 69 bp, Artificial Sequence
  cDNA Sequence of aMTD685 5'-primer
gggtttcatatggcgctgctggtggcggtgctgccggcggcgctgccggcaaatattaccgttttctat

SEQ ID NO: 693 - DNA, 69 bp, Artificial Sequence
  cDNA Sequence of aMTD686 5'-primer
gggtttcatatggcggcgctggtggcggtgctgccggtggcgctgccggcaaatattaccgttttctat

SEQ ID NO: 694 - DNA, 69 bp, Artificial Sequence
  cDNA Sequence of aMTD687 5'-primer
gggtttcatatggcgattctggcggtggcgctgccgctgctggcgccggcaaatattaccgttttctat

SEQ ID NO: 695 - DNA, 69 bp, Artificial Sequence
  cDNA Sequence of aMTD692 5'-primer
gggtttcatatgccggcgccgctgccgccggtggtgattctggcggtggcaaatattaccgttttctat

SEQ ID NO: 696 - DNA, 69 bp, Artificial Sequence
  cDNA Sequence of aMTD693 5'-primer
gggtttcatatggcggcgccggtgctgccggtggcggtgccgattgtggcaaatattaccgttttctat

SEQ ID NO: 697 - DNA, 69 bp, Artificial Sequence
  cDNA Sequence of aMTD700 5'-primer
gggtttcatatgggcaccagcaacacctgccagagcaaccagaacagcgcaaatattaccgttttctat

SEQ ID NO: 698 - DNA, 69 bp, Artificial Sequence
  cDNA Sequence of aMTD703 5'-primer
gggtttcatatgattgtggcggtggcgctggtgccggcgctggcgccggcaaatattaccgttttctat

SEQ ID NO: 699 - DNA, 68 bp, Artificial Sequence
  cDNA Sequence of aMTD705 5'-primer
gggtttcatatattgtggcggtggcgctgctgccggcgctggcgccggcaaatattaccgttttctat

SEQ ID NO: 700 - DNA, 69 bp, Artificial Sequence
  cDNA Sequence of aMTD706 5'-primer
gggtttcatatgattgtggcggtggcgctgctgccggcggtggcgccggcaaatattaccgttttctat

SEQ ID NO: 701 - DNA, 69 bp, Artificial Sequence
  cDNA Sequence of aMTD707 5'-primer
gggtttcatatgattgtggcgctggcggtgctgccggcggtggcgccggcaaatattaccgttttctat

SEQ ID NO: 702 - DNA, 69 bp, Artificial Sequence
  cDNA Sequence of aMTD724 5'-primer
gggtttcatatggtggcggtgctggcggtgctgccggcgctggcgccggcaaatattaccgttttctat

SEQ ID NO: 703 - DNA, 69 bp, Artificial Sequence
  cDNA Sequence of aMTD725 5'-primer
gggtttcatatgattgcggtgctggcggtggcgccggcggtgctgccggcaaatattaccgttttctat

SEQ ID NO: 704 - DNA, 69 bp, Artificial Sequence
  cDNA Sequence of aMTD726 5'-primer
gggtttcatatgctggcggtggcgattattgcgccggcggtggcgccggcaaatattaccgttttctat

SEQ ID NO: 705 - DNA, 69 bp, Artificial Sequence
  cDNA Sequence of aMTD727 5'-primer
gggtttcatatggtggcgctggcgattgcgctgccggcggtgctgccggcaaatattaccgttttctat

SEQ ID NO: 706 - DNA, 69 bp, Artificial Sequence
  cDNA Sequence of aMTD743 5'-primer
gggtttcatatggcgattgcgattgcgctggtgccggtggcgctgccggcaaatattaccgttttctat

SEQ ID NO: 707 - DNA, 69 bp, Artificial Sequence
  cDNA Sequence of aMTD744 5'-primer
gggtttcatatggcggcggtggtgattgtggcgccggtggcgctgccggcaaatattaccgttttctat

SEQ ID NO: 708 - DNA, 69 bp, Artificial Sequence
  cDNA Sequence of aMTD745 5'-primer
gggtttcatatggcggcgattctggcgattgtggcgccgctggcgccggcaaatattaccgttttctat

SEQ ID NO: 709 - DNA, 69 bp, Artificial Sequence
  cDNA Sequence of aMTD746 5'-primer
gggtttcatatggtggcgattattgtggtggcgccggcgctggcgccggcaaatattaccgttttctat

SEQ ID NO: 710 - DNA, 69 bp, Artificial Sequence
  cDNA Sequence of aMTD747 5'-primer
gggtttcatatggtggcgctgctggcgattgcgccggcgctggcgccggcaaatattaccgttttctat

SEQ ID NO: 711 - DNA, 69 bp, Artificial Sequence
  cDNA Sequence of aMTD750 5'-primer
gggtttcatatgctggcgattgcggcgattgcgccgctggcgattccggcaaatattaccgttttctat

SEQ ID NO: 712 - DNA, 69 bp, Artificial Sequence
  cDNA Sequence of aMTD763 5'-primer
gggtttcatatggtggcggtgctgattgcggtgccggcgctggcgccggcaaatattaccgttttctat

SEQ ID NO: 713 - DNA, 69 bp, Artificial Sequence
  cDNA Sequence of aMTD764 5'-primer
gggtttcatatggcggtggcgctggcggtgctgccggcggtggtgccggcaaatattaccgttttctat

SEQ ID NO: 714 - DNA, 69 bp, Artificial Sequence
  cDNA Sequence of aMTD765 5'-primer
gggtttcatatggcggtggcgctggcggtggtgccggcggtgctgccggcaaatattaccgttttctat

SEQ ID NO: 715 - DNA, 69 bp, Artificial Sequence
  cDNA Sequence of aMTD766 5'-primer
gggtttcatatgattgtggtgattgcggtggcgccggcggtggcgccggcaaatattaccgttttctat

SEQ ID NO: 716 - DNA, 69 bp, Artificial Sequence
  cDNA Sequence of aMTD767 5'-primer
gggtttcatatgattgtggtggcggcggtggtgccggcgctggcgccggcaaatattaccgttttctat

SEQ ID NO: 717 - DNA, 69 bp, Artificial Sequence
  cDNA Sequence of aMTD772 5'-primer
gggtttcatatgctgccggtggcgccggtgattccgattattgtgccggcaaatattaccgttttctat

SEQ ID NO: 718 - DNA, 69 bp, Artificial Sequence
  cDNA Sequence of aMTD783 5'-primer
gggtttcatatgattgtggcgctggtgccggcggtggcgattgcgccggcaaatattaccgttttctat

SEQ ID NO: 719 - DNA, 69 bp, Artificial Sequence
  cDNA Sequence of aMTD784 5'-primer
gggtttcatatggtggcggcgctgccggcggtggcgctggtggtgccggcaaatattaccgttttctat

SEQ ID NO: 720 - DNA, 69 bp, Artificial Sequence
  cDNA Sequence of aMTD786 5'-primer
gggtttcatatgctggtggcgattgcgccgctggcggtgctggcgccggcaaatattaccgttttctat

SEQ ID NO: 721 - DNA, 69 bp, Artificial Sequence
  cDNA Sequence of aMTD787 5'-primer
gggtttcatatggcggtggcgctggtgccggtgattgtggcggcgccggcaaatattaccgttttctat

SEQ ID NO: 722 - DNA, 69 bp, Artificial Sequence
  cDNA Sequence of aMTD788 5'-primer
gggtttcatatggcgattgcggtggcgattgcgccggtggcgctgccggcaaatattaccgttttctat

SEQ ID NO: 723 - DNA, 69 bp, Artificial Sequence
  cDNA Sequence of aMTD803 5'-primer
gggtttcatatggcgattgcgctggcggtgccggtgctggcgctgccggcaaatattaccgttttctat

SEQ ID NO: 724 - DNA, 69 bp, Artificial Sequence
  cDNA Sequence of aMTD805 5'-primer
gggtttcatatgctggtgctgattgcggcggcgccgattgcgctgccggcaaatattaccgttttctat

SEQ ID NO: 725 - DNA, 69 bp, Artificial Sequence
  cDNA Sequence of aMTD806 5'-primer
gggtttcatatgctggtggcgctggcggtgccggcggcggtgctgccggcaaatattaccgttttctat

SEQ ID NO: 726 - DNA, 69 bp, Artificial Sequence
  cDNA Sequence of aMTD807 5'-primer
gggtttcatatggcggtggcgctggcggtgccggcgctggtgctgccggcaaatattaccgttttctat

SEQ ID NO: 727 - DNA, 69 bp, Artificial Sequence
  cDNA Sequence of aMTD808 5'-primer
gggtttcatatgctggtggtgctggcggcggcgccgctggcggtgccggcaaatattaccgttttctat

SEQ ID NO: 728 - DNA, 69 bp, Artificial Sequence
  cDNA Sequence of aMTD809 5'-primer
gggtttcatatgctgattgtgctggcggcgccggcgctggcggcgccggcaaatattaccgttttctat

SEQ ID NO: 729 - DNA, 69 bp, Artificial Sequence
  cDNA Sequence of aMTD810 5'-primer
gggtttcatatggtgattgtgctggcggcgccggcgctggcggcgccggcaaatattaccgttttctat

SEQ ID NO: 730 - DNA, 69 bp, Artificial Sequence
  cDNA Sequence of aMTD811 5'-primer
gggtttcatatggcggtggtgctggcggtgccggcgctggcggtgccggcaaatattaccgttttctat

SEQ ID NO: 731 - DNA, 69 bp, Artificial Sequence
  cDNA Sequence of aMTD824 5'-primer
gggtttcatatgctgattattgtggcggcggcgccggcggtggcgccggcaaatattaccgttttctat

SEQ ID NO: 732 - DNA, 69 bp, Artificial Sequence
  cDNA Sequence of aMTD825 5'-primer
gggtttcatatgattgtggcggtgattgtggcgccggcggtggcgccggcaaatattaccgttttctat

SEQ ID NO: 733 - DNA, 69 bp, Artificial Sequence
  cDNA Sequence of aMTD826 5'-primer
gggtttcatatgctggtggcgctggcggcgccgattattgcggtgccggcaaatattaccgttttctat

SEQ ID NO: 734 - DNA, 69 bp, Artificial Sequence
  cDNA Sequence of aMTD827 5'-primer
gggtttcatatgattgcggcggtgctggcggcgccggcgctggtgccggcaaatattaccgttttctat

SEQ ID NO: 735 - DNA, 69 bp, Artificial Sequence
  cDNA Sequence of aMTD828 5'-primer
gggtttcatatgattgcgctgctggcggcgccgattattgcggtgccggcaaatattaccgttttctat

SEQ ID NO: 736 - DNA, 69 bp, Artificial Sequence
  cDNA Sequence of aMTD829 5'-primer
gggtttcatatggcggcgctggcgctggtggcgccggtgattgtgccggcaaatattaccgttttctat

SEQ ID NO: 737 - DNA, 69 bp, Artificial Sequence
  cDNA Sequence of aMTD830 5'-primer
gggtttcatatgattgcgctggtggcggcgccggtggcgctggtgccggcaaatattaccgttttctat

SEQ ID NO: 738 - DNA, 69 bp, Artificial Sequence
  cDNA Sequence of aMTD831 5'-primer
gggtttcatatgattattgtggcggtggcgccggcggcgattgtgccggcaaatattaccgttttctat

SEQ ID NO: 739 - DNA, 69 bp, Artificial Sequence
  cDNA Sequence of aMTD832 5'-primer
gggtttcatatggcggtggcggcgattgtgccggtgattgtggcgccggcaaatattaccgttttctat

SEQ ID NO: 740 - DNA, 69 bp, Artificial Sequence
  cDNA Sequence of aMTD843 5'-primer
gggtttcatatggcggtgctggtgctggtggcgccggcggcggcgccggcaaatattaccgttttctat

SEQ ID NO: 741 - DNA, 69 bp, Artificial Sequence
  cDNA Sequence of aMTD844 5'-primer
gggtttcatatggtggtggcgctgctggcgccgctgattgcggcgccggcaaatattaccgttttctat

SEQ ID NO: 742 - DNA, 69 bp, Artificial Sequence
  cDNA Sequence of aMTD845 5'-primer
gggtttcatatggcggcggtggtgattgcgccgctgctggcggtgccggcaaatattaccgttttctat

SEQ ID NO: 743 - DNA, 69 bp, Artificial Sequence
  cDNA Sequence of aMTD846 5'-primer
gggtttcatatgattgcggtggcggtggcggcgccgctgctggtgccggcaaatattaccgttttctat

SEQ ID NO: 744 - DNA, 69 bp, Artificial Sequence
  cDNA Sequence of aMTD847 5'-primer
gggtttcatatgctggtggcgattgtggtgctgccggcggtggcgccggcaaatattaccgttttctat

SEQ ID NO: 745 - DNA, 69 bp, Artificial Sequence
  cDNA Sequence of aMTD848 5'-primer
gggtttcatatggcggtggcgattgtggtgctgccggcggtggcgccggcaaatattaccgttttctat

SEQ ID NO: 746 - DNA, 69 bp, Artificial Sequence
  cDNA Sequence of aMTD849 5'-primer
gggtttcatatggcggtgattctgctggcgccgctgattgcggcgccggcaaatattaccgttttctat

SEQ ID NO: 747 - DNA, 69 bp, Artificial Sequence
  cDNA Sequence of aMTD850 5'-primer
gggtttcatatgctggtgattgcgctggcggcgccggtggcgctgccggcaaatattaccgttttctat

SEQ ID NO: 748 - DNA, 69 bp, Artificial Sequence
  cDNA Sequence of aMTD851 5'-primer
gggtttcatatggtgctggcggtggtgctgccggcggtggcgctgccggcaaatattaccgttttctat

SEQ ID NO: 749 - DNA, 69 bp, Artificial Sequence
  cDNA Sequence of aMTD852 5'-primer
gggtttcatatggtgctggcggtggcggcgccggcggtgctgctgccggcaaatattaccgttttctat

SEQ ID NO: 750 - DNA, 69 bp, Artificial Sequence
  cDNA Sequence of aMTD863 5'-primer
gggtttcatatggcggcggtggtgctgctgccgattattgcggcgccggcaaatattaccgttttctat

SEQ ID NO: 751 - DNA, 69 bp, Artificial Sequence
  cDNA Sequence of aMTD864 5'-primer
gggtttcatatggcgctgctggtgattgcgccggcgattgcggtgccggcaaatattaccgttttctat

SEQ ID NO: 752 - DNA, 69 bp, Artificial Sequence
  cDNA Sequence of aMTD865 5'-primer
gggtttcatatggcggtgctggtgattgcggtgccggcgattgcgccggcaaatattaccgttttctat

SEQ ID NO: 753 - DNA, 69 bp, Artificial Sequence
  cDNA Sequence of aMTD867 5'-primer
gggtttcatatggcgctgctggtggtgattgcgccgctggcggcgccggcaaatattaccgttttctat

SEQ ID NO: 754 - DNA, 69 bp, Artificial Sequence
  cDNA Sequence of aMTD868 5'-primer
gggtttcatatggtgctggtggcggcgattctgccggcggcgattccggcaaatattaccgttttctat

SEQ ID NO: 755 - DNA, 69 bp, Artificial Sequence
  cDNA Sequence of aMTD870 5'-primer
gggtttcatatggtgctggtggcggcggtgctgccgattgcggcgccggcaaatattaccgttttctat

SEQ ID NO: 756 - DNA, 69 bp, Artificial Sequence
  cDNA Sequence of aMTD872 5'-primer
gggtttcatatggtgctggcggcggcggtgctgccgctggtggtgccggcaaatattaccgttttctat

SEQ ID NO: 757 - DNA, 69 bp, Artificial Sequence
  cDNA Sequence of aMTD875 5'-primer
gggtttcatatggcgattgcgattgtggtgccggcggtggcggtgccggcaaatattaccgttttctat

SEQ ID NO: 758 - DNA, 69 bp, Artificial Sequence
  cDNA Sequence of aMTD877 5'-primer
gggtttcatatggtggcgattattgcggtgccggcggtggtggcgccggcaaatattaccgttttctat

SEQ ID NO: 759 - DNA, 69 bp, Artificial Sequence
  cDNA Sequence of aMTD878 5'-primer
gggtttcatatgattgtggcgctggtggcgccggcggcggtggtgccggcaaatattaccgttttctat

SEQ ID NO: 760 - DNA, 69 bp, Artificial Sequence
  cDNA Sequence of aMTD879 5'-primer
gggtttcatatggcggcgattgtgctgctgccggcggtggtggtgccggcaaatattaccgttttctat

SEQ ID NO: 761 - DNA, 69 bp, Artificial Sequence
  cDNA Sequence of aMTD881 5'-primer
gggtttcatatggcggcgctgattgtggtgccggcggtggcggtgccggcaaatattaccgttttctat

SEQ ID NO: 762 - DNA, 69 bp, Artificial Sequence
  cDNA Sequence of aMTD882 5'-primer
gggtttcatatggcgattgcgctggtggtgccggcggtggcggtgccggcaaatattaccgttttctat

SEQ ID NO: 763 - DNA, 69 bp, Artificial Sequence
  cDNA Sequence of aMTD883 5'-primer
gggtttcatatgctggcgattgtgccggcggcgattgcggcgctgccggcaaatattaccgttttctat

SEQ ID NO: 764 - DNA, 69 bp, Artificial Sequence
  cDNA Sequence of aMTD884 5'-primer
gggtttcatatggtgctgattgtgccggcggcgattgcggcgctgccggcaaatattaccgttttctat

SEQ ID NO: 765 - DNA, 69 bp, Artificial Sequence
  cDNA Sequence of aMTD885 5'-primer
gggtttcatatgctggtggcgattgcgccggcggtggcggtgctgccggcaaatattaccgttttctat

SEQ ID NO: 766 - DNA, 69 bp, Artificial Sequence
  cDNA Sequence of aMTD886 5'-primer
gggtttcatatggtgctggcggtgccggcggcgattgcggcgctgccggcaaatattaccgttttctat

SEQ ID NO: 767 - DNA, 69 bp, Artificial Sequence
  cDNA Sequence of aMTD887 5'-primer
gggtttcatatggtgctggcggtggcgccggcggtggcggtgctgccggcaaatattaccgttttctat

SEQ ID NO: 768 - DNA, 69 bp, Artificial Sequence
  cDNA Sequence of aMTD888 5'-primer
gggtttcatatgattctggcggtggtggcgattccggcggcggcgccggcaaatattaccgttttctat

SEQ ID NO: 769 - DNA, 69 bp, Artificial Sequence
  cDNA Sequence of aMTD889 5'-primer
gggtttcatatgattctggtggcggcggcgccgattgcggcgctgccggcaaatattaccgttttctat

SEQ ID NO: 770 - DNA, 69 bp, Artificial Sequence
  cDNA Sequence of aMTD891 5'-primer
gggtttcatatgattctggcggtggcggcgattccggcggcgctgccggcaaatattaccgttttctat

SEQ ID NO: 771 - DNA, 69 bp, Artificial Sequence
  cDNA Sequence of aMTD893 5'-primer
gggtttcatatggtgattgcgattccggcgattctggcggcggcgccggcaaatattaccgttttctat

SEQ ID NO: 772 - DNA, 69 bp, Artificial Sequence
  cDNA Sequence of aMTD895 5'-primer
gggtttcatatggcgattattattgtggtgccggcgattgcggcgccggcaaatattaccgttttctat

SEQ ID NO: 773 - DNA, 69 bp, Artificial Sequence
  cDNA Sequence of aMTD896 5'-primer
gggtttcatatggcgattctgattgtggtggcgccgattgcggcgccggcaaatattaccgttttctat

SEQ ID NO: 774 - DNA, 69 bp, Artificial Sequence
  cDNA Sequence of aMTD897 5'-primer
gggtttcatatggcggtgattgtgccggtggcgattattgcggcgccggcaaatattaccgttttctat

SEQ ID NO: 775 - DNA, 69 bp, Artificial Sequence
  cDNA Sequence of aMTD899 5'-primer
gggtttcatatggcggtggtgattgcgctgccggcggtggtggcgccggcaaatattaccgttttctat

SEQ ID NO: 776 - DNA, 69 bp, Artificial Sequence
  cDNA Sequence of aMTD900 5'-primer
gggtttcatatggcgctggtggcggtgattgcgccggtggtggcgccggcaaatattaccgttttctat

SEQ ID NO: 777 - DNA, 69 bp, Artificial Sequence
  cDNA Sequence of aMTD901 5'-primer
gggtttcatatggcgctggtggcggtgctgccggcggtggcggtgccggcaaatattaccgttttctat

SEQ ID NO: 778 - DNA, 69 bp, Artificial Sequence
  cDNA Sequence of aMTD902 5'-primer
gggtttcatatggcgctggtggcgccgctgctggcggtggcggtgccggcaaatattaccgttttctat

SEQ ID NO: 779 - DNA, 69 bp, Artificial Sequence
  cDNA Sequence of aMTD904 5'-primer
gggtttcatatggcggtgctggcggtggtggcgccggtggtggcgccggcaaatattaccgttttctat

SEQ ID NO: 780 - DNA, 69 bp, Artificial Sequence
  cDNA Sequence of aMTD905 5'-primer
gggtttcatatggcggtgattgcggtggcgccgctggtggtggcgccggcaaatattaccgttttctat

SEQ ID NO: 781 - DNA, 69 bp, Artificial Sequence
  cDNA Sequence of aMTD906 5'-primer
gggtttcatatggcggtgattgcgctggcgccggtggtggtggcgccggcaaatattaccgttttctat

SEQ ID NO: 782 - DNA, 69 bp, Artificial Sequence
  cDNA Sequence of aMTD907 5'-primer
gggtttcatatggtggcgattgcgctggcgccggtggtggtggcgccggcaaatattaccgttttctat

SEQ ID NO: 783 - DNA, 69 bp, Artificial Sequence
  cDNA Sequence of aMTD908 5'-primer
gggtttcatatggtggcgctggcgctggcgccggtggtggtggcgccggcaaatattaccgttttctat

SEQ ID NO: 784 - DNA, 69 bp, Artificial Sequence
  cDNA Sequence of aMTD910 5'-primer
gggtttcatatggtggcggcgctgctgccggcggtggtggtggcgccggcaaatattaccgttttctat

SEQ ID NO: 785 - DNA, 69 bp, Artificial Sequence
  cDNA Sequence of aMTD911 5'-primer
gggtttcatatggtggcgctggcgctgccggcggtggtggtggcgccggcaaatattaccgttttctat

SEQ ID NO: 786 - DNA, 69 bp, Artificial Sequence
  cDNA Sequence of aMTD912 5'-primer
gggtttcatatggtggcgctgctggcgccggcggtggtggtggcgccggcaaatattaccgttttctat

SEQ ID NO: 787 - DNA, 69 bp, Artificial Sequence
  cDNA Sequence of aMTD921 5'-primer
gggtttcatatgatttggtggtttgtggtgctgccgctggtggtgccggcaaatattaccgttttctat

SEQ ID NO: 788 - DNA, 69 bp, Artificial Sequence
  cDNA Sequence of aMTD922 5'-primer
gggtttcatatgtggtatgtgatttttgtgctgccgctggtggtgccggcaaatattaccgttttctat

SEQ ID NO: 789 - DNA, 69 bp, Artificial Sequence
  cDNA Sequence of aMTD931 5'-primer
gggtttcatatggcggtgctgattgcgccggcgattctggcggcggcggcaaatattaccgttttctat

SEQ ID NO: 790 - DNA, 69 bp, Artificial Sequence
  cDNA Sequence of aMTD934 5'-primer
gggtttcatatgctgattctggcgccggcggcggtggtggcggcggcggcaaatattaccgttttctat

SEQ ID NO: 791 - DNA, 69 bp, Artificial Sequence
  cDNA Sequence of aMTD935 5'-primer
gggtttcatatggcgctgctgattctgccggcggcggcggtggcggcggcaaatattaccgttttctat

SEQ ID NO: 792 - DNA, 69 bp, Artificial Sequence
  cDNA Sequence of aMTD936 5'-primer
gggtttcatatggcgctgctgattctggcggcggcggtggcggcgccggcaaatattaccgttttctat

SEQ ID NO: 793 - DNA, 69 bp, Artificial Sequence
  cDNA Sequence of aMTD937 5'-primer
gggtttcatatggtgccggtgctggtgccgctgccggtgccggtggtggcaaatattaccgttttctat

SEQ ID NO: 794 - DNA, 69 bp, Artificial Sequence
  cDNA Sequence of aMTD938 5'-primer
gggtttcatatggtgccggtgctgctgccggtggtggtgccggtgccggcaaatattaccgttttctat

SEQ ID NO: 795 - DNA, 69 bp, Artificial Sequence
  cDNA Sequence of aMTD947 5'-primer
gggtttcatatgtgctattataatcagcagtccaataataataatcaggcaaatattaccgttttctat

SEQ ID NO: 796 - DNA, 69 bp, Artificial Sequence
  cDNA Sequence of aMTD949 5'-primer
gggtttcatatgtccggcaattcctgccagcagtgcggcaattcctccgcaaatattaccgttttctat

SEQ ID NO: 797 - DNA, 39 bp, Artificial Sequence
  cDNA Sequence of aMTD 3'-primer
cgcgtcgacttacctcggctgcaccggcacggagatgac

SEQ ID NO: 798 - protein, 184 aa, Artificial Sequence
  Amino acid Sequence of SDA
MANITVFYNEDFQGKQVDLPPGNYTRAQLAALGIENNTISSVKVPPGVKAILYQNDGFAGDQIEVVANAEELGPLNNNVSSIRVISVPVQPRMANITVFYNEDFQGKQVDLPPGNYTRAQLAALGIENNTISSVKVPPGVKAILYQNDGFAGDQIEVVANAEELGPLNNNVSSIRVISVPVQPR

SEQ ID NO: 799 - protein, 99 aa, Artificial Sequence
  Amino acid Sequence of SDB
MAEQSDKDVKYYTLEEIQKHKDSKSTWVILHHKVYDLTKFLEEHPGGEEVLGEQAGGDATENFEDVGHSTDARELSKTYIIGELHPDDRSKIAKPSETL

SEQ ID NO: 800 - protein, 109 aa, Artificial Sequence
  Amino acid Sequence of SDC
MSDKIIHLTDDSFDTDVLKADGAILVDFWAEWCGPCKMIAPILDEIADEYQGKLTVAKLNIDQNPGTAPKYGIRGIPTLLLFKNGEVAATKVGALSKGQLKEFLDANLA

SEQ ID NO: 801 - protein, 208 aa, Artificial Sequence
  Amino acid Sequence of SDD
MKKIWLALAGLVLAFSASAAQYEDGKQYTTLEKPVAGAPQVLEFFSFFCPHCYQFEEVLHISDNVKKKLPEGVKMTKYHVNFMGGDLGKDLTQAWAVAMALGVEDKVTVPLFEGVQKTQTIRSASDIRDVFINAGIKGEEYDAAWNSFVVKSLVAQQEKAAADVQLRGVPAMFVNGKYQLNPQGMDTSNMDVFVQQYADTVKYLSEKK

SEQ ID NO: 802 - protein, 100 aa, Artificial Sequence
  Amino acid Sequence of SDE
GSLQDSEVNQEAKPEVKPEVKPETHINLKVSDGSSEIFFKIKKTTPLRRLMEAFAKRQGKEMDSLTFLYDGIEIQADQTPEDLDMEDNDIIEAHREQIGG

SEQ ID NO: 803 - protein, 297 aa, Artificial Sequence
  Amino acid Sequence of SDF
GSEIGTGFPFDPHYVEVLGERMHYVDVGPRDGTPVLFLHGNPTSSYVWRNIIPHVAPTHRCIAPDLIGMGKSDKPDLGYFFDDHVRFMDAFIEALGLEEVVLVIHDWGSALGFHWAKRNPERVKGIAFMEFIRPIPTWDEWPEFARETFQAFRTTDVGRKLIIDQNVFIEGTLPMGVVRPLTEVEMDHYREPFLNPVDREPLWRFPNELPIAGEPANIVALVEEYMDWLHQSPVPKLLFWGTPGVLIPPAEAARLAKSLPNCKAVDIGPGLNLLQEDNPDLIGSEIARWLSTLEISG

SEQ ID NO: 804 - protein, 99 aa, Artificial Sequence
  Amino acid Sequence of SDB' for deimunization
MAEQSDKDVKYYTLEEIQKHKDSKSTWLILHHKVYDLTKFLEEHPGGEEVLGEQAGGDATENFEDVGHSTDARELSKTYIIGELHPDDRSKIAKPSETL

SEQ ID NO: 805 - DNA, 552 bp, Artificial Sequence
  cDNA Sequence of SDA
atggcaaatattaccgttttctataacgaagacttccagggtaagcaggtcgatctgccgcctggcaactatacccgcgcccagttggcggcgctgggcatcgagaataataccatcagctcggtgaaggtgccgcctggcgtgaaggctatcctgtaccagaacgatggtttcgccggcgaccagatcgaagtggtggccaatgccgaggagttgggcccgctgaataataacgtctccagcatccgcgtcatctccgtgcccgtgcagccgcgcatggcaaatattaccgttttctataacgaagacttccagggtaagcaggtcgatctgccgcctggcaactatacccgcgcccagttggcggcgctgggcatcgagaataataccatcagctcggtgaaggtgccgcctggcgtgaaggctatcctctaccagaacgatggtttcgccggcgaccagatcgaagtggtggccaatgccgaggagctgggtccgctgaataataacgtctccagcatccgcgtcatctccgtgccggtgcagccgagg

SEQ ID NO: 806 - DNA, 297 bp, Artificial Sequence
  cDNA Sequence of SDB
atggcagaacaaagcgacaaggatgtgaagtactacactctggaggagattcagaagcacaaagacagcaagagcacctgggtgatcctacatcataaggtgtacgatctgaccaagtttctcgaagagcatcctggtggggaagaagtcctgggcgagcaagctgggggtgatgctactgagaactttgaggacgtcgggcactctacggatgcacgagaactgtccaaaacatacatcatcggggagctccatccagatgacagatcaaagatagccaagccttcggaaaccctt

SEQ ID NO: 807 - DNA, 327 bp, Artificial Sequence
  cDNA Sequence of SDC
atgagcgataaaattattcacctgactgacgacagttttgacacggatgtactcaaagcggacggggcgatcctcgtcgatttctgggcagagtggtgcggtccgtgcaaaatgatcgccccgattctggatgaaatcgctgacgaatatcagggcaaactgaccgttgcaaaactgaacatcgatcaaaaccctggcactgcgccgaaatatggcatccgtggtatcccgactctgctgctgttcaaaaacggtgaagtggcggcaaccaaagtgggtgcactgtctaaaggtcagttgaaagagttcctcgacgctaacctggcc

SEQ ID NO: 808 - DNA, 624 bp, Artificial Sequence
  cDNA Sequence of SDD
atgaaaaagatttggctggcgctggctggtttagttttagcgtttagcgcatcggcggcgcagtatgaagatggtaaacagtacactaccctggaaaaaccggtagctggcgcgccgcaagtgctggagtttttctctttcttctgcccgcactgctatcagtttgaagaagttctgcatatttctgataatgtgaagaaaaaactgccggaaggcgtgaagatgactaaataccacgtcaacttcatgggtggtgacctgggcaaagatctgactcaggcatgggctgtggcgatggcgctgggcgtggaagacaaagtgactgttccgctgtttgaaggcgtacagaaaacccagaccattcgttctgcttctgatatccgcgatgtatttatcaacgcaggtattaaaggtgaagagtacgacgcggcgtggaacagcttcgtggtgaaatctctggtcgctcagcaggaaaaagctgcagctgacgtgcaattgcgtggcgttccggcgatgtttgttaacggtaaatatcagctgaatccgcagggtatggataccagcaatatggatgtttttgttcagcagtatgctgatacagtgaaatatctgtccgagaaaaaa

SEQ ID NO: 809 - DNA, 300 bp, Artificial Sequence
  cDNA Sequence of SDE
gggtccctgcaggactcagaagtcaatcaagaagctaagccagaggtcaagccagaagtcaagcctgagactcacatcaatttaaaggtgtccgatggatcttcagagatcttcttcaagatcaaaaagaccactcctttaagaaggctgatggaagcgttcgctaaaagacagggtaaggaaatggactccttaacgttcttgtacgacggtattgaaattcaagctgatcagacccctgaagatttggacatggaggataacgatattattgaggctcaccgcgaacagattggaggt

SEQ ID NO: 810 - DNA, 891 bp, Artificial Sequence
  cDNA Sequence of SDF
ggatccgaaatcggtactggctttccattcgacccccattatgtggaagtcctgggcgagcgcatgcactacgtcgatgttggtccgcgcgatggcacccctgtgctgttcctgcacggtaacccgacctcctcctacgtgtggcgcaacatcatcccgcatgttgcaccgacccatcgctgcattgctccagacctgatcggtatgggcaaatccgacaaaccagacctgggttatttcttcgacgaccacgtccgcttcatggatgccttcatcgaagccctgggtctggaagaggtcgtcctggtcattcacgactggggctccgctctgggtttccactgggccaagcgcaatccagagcgcgtcaaaggtattgcatttatggagttcatccgccctatcccgacctgggacgaatggccagaatttgcccgcgagaccttccaggccttccgcaccaccgacgtcggccgcaagctgatcatcgatcagaacgtttttatcgagggtacgctgccgatgggtgtcgtccgcccgctgactgaagtcgagatggaccattaccgcgagccgttcctgaatcctgttgaccgcgagccactgtggcgcttcccaaacgagctgccaatcgccggtgagccagcgaacatcgtcgcgctggtcgaagaatacatggactggctgcaccagtcccctgtcccgaagctgctgttctggggcaccccaggcgttctgatcccaccggccgaagccgctcgcctggccaaaagcctgcctaactgcaaggctgtggacatcggcccgggtctgaatctgctgcaagaagacaacccggacctgatcggcagcgagatcgcgcgctggctgtctactctggagatttccggt

SEQ ID NO: 811 - DNA, 297 bp, Artificial Sequence
  cDNA Sequence of SDB' for deimunization
atggcagaacaaagcgacaaggatgtgaagtactacactctggaggagattcagaagcacaaagacagcaagagcacctggctgatcctacatcataaggtgtacgatctgaccaagtttctcgaagagcatcctggtggggaagaagtcctgggcgagcaagctgggggtgatgctactgagaactttgaggacgtcgggcactctacggatgcacgagaactgtccaaaacatacatcatcggggagctccatccagatgacagatcaaagatagccaagccttcggaaaccctt

SEQ ID NO: 812 - protein, 19 aa, Artificial Sequence
  Amino acid Sequence of Histidine Tag
MGSSHHHHHHSSGLVPRGS

SEQ ID NO: 813 - DNA, 57 bp, Artificial Sequence
  cDNA Sequence of Histidine Tag
atgggcagcagccatcatcatcatcatcacagcagcggcctggtgccgcgcggcagc

SEQ ID NO: 814 - protein, 225 aa, Artificial Sequence
  Amino Acid Sequence of Human SOCS3
MVTHSKFPAAGMSRPLDTSLRLKTFSSKSEYQLVVNAVRKLQESGFYWSAVTGGEANLLLSAEPAGTFLIRDSSDQRHFFTLSVKTQSGTKNLRIQCEGGSFSLQSDPRSTQPVPRFDCVLKLVHHYMPPPGAPSFPSPPTEPSSEVPEQPSAQPLPGSPPRRAYYIYSGGEKIPLVLSRPLSSNVATLQHLCRKTVNGHLDSYEKVTQLPGPIREFLDQYDAPL

SEQ ID NO: 815 - DNA, 675 bp, Artificial Sequence
  cDNA Sequences of Human SOCS3
atggtcacccacagcaagtttcccgccgccgggatgagccgccccctggacaccagcctgcgcctcaagaccttcagctccaagagcgagtaccagctggtggtgaacgcagtgcgcaagctgcaggagagcggcttctactggagcgcagtgaccggcggcgaggcgaacctgctgctcagtgccgagcccgccggcacctttctgatccgcgacagctcggaccagcgccacttcttcacgctcagcgtcaagacccagtctgggaccaagaacctgcgcatccagtgtgaggggggcagcttctctctgcagagcgatccccggagcacgcagcccgtgccccgcttcgactgcgtgctcaagctggtgcaccactacatgccgccccctggagccccctccttcccctcgccacctactgaaccctcctccgaggtgcccgagcagccgtctgcccagccactccctgggagtccccccagaagagcctattacatctactccgggggcgagaagatccccctggtgttgagccggcccctctcctccaacgtggccactcttcagcatctctgtcggaagaccgtcaacggccacctggactcctatgagaaagtcacccagctgccggggcccattcgggagttcctggaccagtacgatgccccgctt

SEQ ID NO: 816 - DNA, 25 bp, Artificial Sequence
  Unmethyl-F primer
tagtgtgtaagttgtaggagagtgg

SEQ ID NO: 817 - DNA, 30 bp, Artificial Sequence
  Unmethyl-R primer
ctaaacataaaaaaataacactaatccaaa

SEQ ID NO: 818 - DNA, 24 bp, Artificial Sequence
  Methyl-F primer
gtagtgcgtaagttgtaggagagc

SEQ ID NO: 819 - DNA, 24 bp, Artificial Sequence
  Methyl-R primer
gtaaaaaaataacgctaatccgaa

SEQ ID NO: 820 - DNA, 20 bp, Artificial Sequence
  SOCS3 primer F
cctactgaaccctcctccga

SEQ ID NO: 821 - DNA, 20 bp, Artificial Sequence
  SOCS3 primer R
gcagctgggtgactttctca

SEQ ID NO: 822 - protein, 12 aa, Artificial Sequence
  Amino acid Sequence of aMTD662
ALAVILAPVAVP

SEQ ID NO: 823 - DNA, 36 bp, Artificial Sequence
  cDNA Sequence of aMTD662
gcgctggcggtgattctggcgccggtggcggtgccg

SEQ ID NO: 824 - DNA, 1005 bp, Artificial Sequence
  cDNA sequence of E.coli codon usage optimized M165S3B'
gcgctggcggtgccggttgcgctggcgatcgtgccggttacccacagcaagtttccggcggcgggtatgagccgtccgctggacaccagcctgcgtctgaagacctttagcagcaaaagcgagtaccagctggttgtgaacgcggtgcgtaaactgcaagaaagcggcttctattggagcgcggttaccggtggcgaggcgaacctgctgctgagcgcggagccggcgggcaccttcctgatccgtgacagcagcgatcagcgtcacttctttaccctgagcgttaagacccagagcggcaccaaaaacctgcgtattcaatgcgagggtggcagcttcagcctgcaaagcgacccgcgtagcacccaaccggtgccgcgttttgattgcgtgctgaagctggttcaccactacatgccgccgccgggtgcgccgagcttcccgagcccgccgaccgagccgagcagcgaggttccggaacagccgagcgcgcaaccgctgccgggtagcccgccgcgtcgtgcgtactatatctatagcggtggcgaaaaaattccgctggtgctgagccgtccgctgagcagcaacgttgcgaccctgcaacacctgtgccgtaagaccgtgaacggtcacctggacagctacgagaaagttacccaactgccgggcccgatccgtgaatttctggaccagtatgatgcgccgctgatggcggaacaaagcgacaaggatgtgaaatactataccctggaggaaatccagaagcacaaagacagcaagagcacctggctgattctgcaccacaaggtgtacgatctgaccaaattcctggaggaacatccgggtggtgaggaagtgctgggcgagcaagcgggtggcgatgcgaccgagaactttgaagacgtgggccacagcaccgatgcgcgtgagctgagcaaaacctatatcattggtgaactgcacccggacgatcgtagcaagattgcgaaaccgagcgaaaccctg

SEQ ID NO: 825 - protein, 335 aa, Artificial Sequence
  Amino acid sequence of E.coli codon usage optimized M165S3B'
ALAVPVALAIVPVTHSKFPAAGMSRPLDTSLRLKTFSSKSEYQLVVNAVRKLQESGFYWSAVTGGEANLLLSAEPAGTFLIRDSSDQRHFFTLSVKTQSGTKNLRIQCEGGSFSLQSDPRSTQPVPRFDCVLKLVHHYMPPPGAPSFPSPPTEPSSEVPEQPSAQPLPGSPPRRAYYIYSGGEKIPLVLSRPLSSNVATLQHLCRKTVNGHLDSYEKVTQLPGPIREFLDQYDAPLMAEQSDKDVKYYTLEEIQKHKDSKSTWLILHHKVYDLTKFLEEHPGGEEVLGEQAGGDATENFEDVGHSTDARELSKTYIIGELHPDDRSKIAKPSETL

SEQ ID NO: 826 - DNA, 1074 bp, Artificial Sequence
  cDNA sequence of HM165S3B
atgggcagcagccatcatcatcatcatcacagcagcggcctggtgccgcgcggcagccatatggcgctggcggtgccggtggcgctggcgattgtgccggtcacccacagcaagtttcccgccgccgggatgagccgccccctggacaccagcctgcgcctcaagaccttcagctccaagagcgagtaccagctggtggtgaacgcagtgcgcaagctgcaggagagcggcttctactggagcgcagtgaccggcggcgaggcgaacctgctgctcagtgccgagcccgccggcacctttctgatccgcgacagctcggaccagcgccacttcttcacgctcagcgtcaagacccagtctgggaccaagaacctgcgcatccagtgtgaggggggcagcttctctctgcagagcgatccccggagcacgcagcccgtgccccgcttcgactgcgtgctcaagctggtgcaccactacatgccgccccctggagccccctccttcccctcgccacctactgaaccctcctccgaggtgcccgagcagccgtctgcccagccactccctgggagtccccccagaagagcctattacatctactccgggggcgagaagatccccctggtgttgagccggcccctctcctccaacgtggccactcttcagcatctctgtcggaagaccgtcaacggccacctggactcctatgagaaagtcacccagctgccggggcccattcgggagttcctggaccagtacgatgccccgcttggatccatggcagaacaaagcgacaaggatgtgaagtactacactctggaggagattcagaagcacaaagacagcaagagcacctgggtgatcctacatcataaggtgtacgatctgaccaagtttctcgaagagcatcctggtggggaagaagtcctgggcgagcaagctgggggtgatgctactgagaactttgaggacgtcgggcactctacggatgcacgagaactgtccaaaacatacatcatcggggagctccatccagatgacagatcaaagatagccaagccttcggaaaccctt

SEQ ID NO: 827 - protein, 362 aa, Artificial Sequence
  Amino acid sequence of HM165S3B
MGSSHHHHHHSSGLVPRGSHMALAVPVALAIVPVTHSKFPAAGMETSRPLDTSLRLKTFSSKSEYQLVVNAVRKLQESGFYWSAVTGGEANLLLSAEPAGTFLIRDSSDQRHFFTLSVKTQSGTKNLRIQCEGGSFSLQSDPRSTQPVPRFDCVLKLVHHYMETPPPGAPSFPSPPTEPSSEVPEQPSAQPLPGSPPRRAYYIYSGGEKIPLVLSRPLSSNVATLQHLCRKTVNGHLDSYEKVTQLPGPIREFLDQYDAPLGSMAEQSDKDVKYYTLEEIQKHKDSKSTWVILHHKVYDLTKFLEEHPGGEEVLGEQAGGDATENFEDVGHSTDARELSKTYIIGELHPDDRSKIAKPSETL

SEQ ID NO: 828 - DNA, 1014 bp, Artificial Sequence
  cDNA sequence of BS3M165
atgatggcagaacaaagcgacaaggatgtgaagtactacactctggaggagattcagaagcacaaagacagcaagagcacctgggtgatcctacatcataaggtgtacgatctgaccaagtttctcgaagagcatcctggtggggaagaagtcctgggcgagcaagctgggggtgatgctactgagaactttgaggacgtcgggcactctacggatgcacgagaactgtccaaaacatacatcatcggggagctccatccagatgacagatcaaagatagccaagccttcggaaacccttggatccgtcacccacagcaagtttcccgccgccgggatgagccgccccctggacaccagcctgcgcctcaagaccttcagctccaagagcgagtaccagctggtggtgaacgcagtgcgcaagctgcaggagagcggcttctactggagcgcagtgaccggcggcgaggcgaacctgctgctcagtgccgagcccgccggcacctttctgatccgcgacagctcggaccagcgccacttcttcacgctcagcgtcaagacccagtctgggaccaagaacctgcgcatccagtgtgaggggggcagcttctctctgcagagcgatccccggagcacgcagcccgtgccccgcttcgactgcgtgctcaagctggtgcaccactacatgccgccccctggagccccctccttcccctcgccacctactgaaccctcctccgaggtgcccgagcagccgtctgcccagccactccctgggagtccccccagaagagcctattacatctactccgggggcgagaagatccccctggtgttgagccggcccctctcctccaacgtggccactcttcagcatctctgtcggaagaccgtcaacggccacctggactcctatgagaaagtcacccagctgccggggcccattcgggagttcctggaccagtacgatgccccgcttccggtgattgcgctggcggtgccggtggcgctggcg

SEQ ID NO: 829 - protein, 342 aa, Artificial Sequence
  Amino acid sequence of BS3M165
MMAEQSDKDVKYYTLEEIQKHKDSKSTWVILHHKVYDLTKFLEEHPGGEEVLGEQAGGDATENFEDVGHSTDARELSKTYIIGELHPDDRSKIAKPSETLGSVTHSKFPAAGMETSRPLDTSLRLKTFSSKSEYQLVVNAVRKLQESGFYWSAVTGGEANLLLSAEPAGTFLIRDSSDQRHFFTLSVKTQSGTKNLRIQCEGGSFSLQSDPRSTQPVPRFDCVLKLVHHYMETPPPGAPSFPSPPTEPSSEVPEQPSAQPLPGSPPRRAYYIYSGGEKIPLVLSRPLSSNVATLQHLCRKTVNGHLDSYEKVTQLPGPIREFLDQYDAPLPVIALAVPVALA

SEQ ID NO: 830 - DNA, 1014 bp, Artificial Sequence
  cDNA sequence of B'S3M165
atgatggcagaacaaagcgacaaggatgtgaagtactacactctggaggagattcagaagcacaaagacagcaagagcacctggctgatcctacatcataaggtgtacgatctgaccaagtttctcgaagagcatcctggtggggaagaagtcctgggcgagcaagctgggggtgatgctactgagaactttgaggacgtcgggcactctacggatgcacgagaactgtccaaaacatacatcatcggggagctccatccagatgacagatcaaagatagccaagccttcggaaacccttggatccgtcacccacagcaagtttcccgccgccgggatgagccgccccctggacaccagcctgcgcctcaagaccttcagctccaagagcgagtaccagctggtggtgaacgcagtgcgcaagctgcaggagagcggcttctactggagcgcagtgaccggcggcgaggcgaacctgctgctcagtgccgagcccgccggcacctttctgatccgcgacagctcggaccagcgccacttcttcacgctcagcgtcaagacccagtctgggaccaagaacctgcgcatccagtgtgaggggggcagcttctctctgcagagcgatccccggagcacgcagcccgtgccccgcttcgactgcgtgctcaagctggtgcaccactacatgccgccccctggagccccctccttcccctcgccacctactgaaccctcctccgaggtgcccgagcagccgtctgcccagccactccctgggagtccccccagaagagcctattacatctactccgggggcgagaagatccccctggtgttgagccggcccctctcctccaacgtggccactcttcagcatctctgtcggaagaccgtcaacggccacctggactcctatgagaaagtcacccagctgccggggcccattcgggagttcctggaccagtacgatgccccgcttccggtgattgcgctggcggtgccggtggcgctggcg

SEQ ID NO: 831 - protein, 342 aa, Artificial Sequence
  Amino acid sequence of B'S3M165
MMAEQSDKDVKYYTLEEIQKHKDSKSTWLILHHKVYDLTKFLEEHPGGEEVLGEQAGGDATENFEDVGHSTDARELSKTYIIGELHPDDRSKIAKPSETLGSVTHSKFPAAGMETSRPLDTSLRLKTFSSKSEYQLVVNAVRKLQESGFYWSAVTGGEANLLLSAEPAGTFLIRDSSDQRHFFTLSVKTQSGTKNLRIQCEGGSFSLQSDPRSTQPVPRFDCVLKLVHHYMETPPPGAPSFPSPPTEPSSEVPEQPSAQPLPGSPPRRAYYIYSGGEKIPLVLSRPLSSNVATLQHLCRKTVNGHLDSYEKVTQLPGPIREFLDQYDAPLPVIALAVPVALA